European Patent Application EP 4 772 613 A1, published July 8, 2026. Title: Chimeric protein or variant thereof comprising IL-2 and IL-15, fusion protein comprising thereof and genetically modified cell. Applicant: GI Cell, Inc. The sequence listing filed with the application follows.

SEQUENCE LISTING (186 sequences)

SEQ ID NO: 1 - protein, 133 aa, Homo sapiens [sequence omitted]

SEQ ID NO: 2 - DNA, 399 bp, Homo sapiens
  source 1..399: mol_type = genomic DNA
gcccccaccagtagcagcaccaagaagacccagcttcagcttgagcatttgcttcttgatctccagatgatactgaatgggatcaacaattataaaaatcctaaattgacacgtatgctgacattcaagttctacatgcctaagaaagcaaccgagcttaaacatttgcagtgcttggaagaagagttgaagcctctcgaggaagtgttgaacttggctcaatccaagaactttcatcttcggcccagagatttgatttcaaatattaacgtcatcgtcctcgagctcaaggggagcgaaaccacattcatgtgtgagtatgcagacgaaaccgccactattgtagaatttcttaatcggtggatcacattctgccaaagcatcatttcaactcttaca

SEQ ID NO: 3 - protein, 23 aa, Homo sapiens
SSTKKTQLQLEHLLLDLQMILNG

SEQ ID NO: 4 - DNA, 69 bp, Homo sapiens
  source 1..69: mol_type = genomic DNA
agctccaccaagaagacacaattgcaactcgaacaccttttgctcgatctgcaaatgatcctcaatggg

SEQ ID NO: 5 - protein, 25 aa, Homo sapiens
INNYKNPKLTRMLTFKFYMPKKATE

SEQ ID NO: 6 - DNA, 75 bp, Homo sapiens
  source 1..75: mol_type = genomic DNA
attaataattacaaaaatcctaaacttactcgcatgttgacattcaagttctatatgccaaaaaaagctaccgag

SEQ ID NO: 7 - protein, 22 aa, Homo sapiens
LKHLQCLEEELKPLEEVLNLAQ

SEQ ID NO: 8 - DNA, 66 bp, Homo sapiens
  source 1..66: mol_type = genomic DNA
ctgaagcacctgcaatgccttgaggaagaactcaaaccattggaagaggttctgaatttggcccag

SEQ ID NO: 9 - protein, 7 aa, Homo sapiens
SKNFHLR

SEQ ID NO: 10 - DNA, 21 bp, Homo sapiens
  source 1..21: mol_type = genomic DNA
tccaaaaactttcatctccga

SEQ ID NO: 11 - protein, 18 aa, Homo sapiens
PRDLISNINVIVLELKGS

SEQ ID NO: 12 - DNA, 54 bp, Homo sapiens
  source 1..54: mol_type = genomic DNA
ccacgagacctcatctctaatattaacgtcattgtacttgagctcaaagggagc

SEQ ID NO: 13 - protein, 14 aa, Homo sapiens
ETTFMCEYADETAT

SEQ ID NO: 14 - DNA, 42 bp, Homo sapiens
  source 1..42: mol_type = genomic DNA
gagaccacctttatgtgcgagtacgccgatgagacagctact

SEQ ID NO: 15 - protein, 20 aa, Homo sapiens
IVEFLNRWITFCQSIISTLT

SEQ ID NO: 16 - DNA, 60 bp, Homo sapiens
  source 1..60: mol_type = genomic DNA
attgttgaattcttgaatagatggattacattttgtcaatctataatctcaaccctgacc

SEQ ID NO: 17 - protein, 133 aa, Homo sapiens
GIHVFILGCFSAGLPKTEANWVNVISDLKKIEDLIQSMHIDATLYTESDVHPSCKVTAMKCFLLELQVISLESGDASIHDTVENLIILANNSLSSNGNVTESGCKECEELEEKNIKEFLQSFVHIVQMFINTS

SEQ ID NO: 18 - DNA, 399 bp, Homo sapiens
  source 1..399: mol_type = genomic DNA
ggcatccacgtgttcattctgggatgcttcagcgcaggcctgcctaaaaccgaggcgaactgggttaacgtgatcagcgatttgaaaaagattgaggatctgatccagtccatgcatattgacgcaaccttgtacacagagtcagatgtgcacccttcctgcaaagttacggctatgaagtgttttttgcttgaattgcaagtaataagtttggagtctggcgatgcatctatacatgataccgtagaaaatttgatcatcctggctaataatagtttgtccagtaatggtaacgtaacagagagcggttgtaaagagtgtgaagagctcgaggaaaagaatataaaagaattcttgcaatcctttgtacatatcgtgcaaatgttcattaatacaagc

SEQ ID NO: 19 - protein, 18 aa, Homo sapiens
ANWVNVISDLKKIEDLIQ

SEQ ID NO: 20 - DNA, 54 bp, Homo sapiens
  source 1..54: mol_type = genomic DNA
gcaaattgggtgaacgtcatatctgaccttaaaaagatagaagacttgatccaa

SEQ ID NO: 21 - protein, 15 aa, Homo sapiens
SMHIDATLYTESDVH

SEQ ID NO: 22 - DNA, 45 bp, Homo sapiens
  source 1..45: mol_type = genomic DNA
agcatgcatatagacgcaacactctacaccgaatccgatgtccat

SEQ ID NO: 23 - protein, 21 aa, Homo sapiens
PSCKVTAMKCFLLELQVISLE

SEQ ID NO: 24 - DNA, 63 bp, Homo sapiens
  source 1..63: mol_type = genomic DNA
ccctcctgcaaggtcaccgccatgaaatgctttctgctcgagttgcaggttattagcctcgaa

SEQ ID NO: 25-26 - skipped (2 entries)

SEQ ID NO: 27 - protein, 20 aa, Homo sapiens
ASIHDTVENLIILANNSLSS

SEQ ID NO: 28 - DNA, 60 bp, Homo sapiens
  source 1..60: mol_type = genomic DNA
gcaagtatccacgatactgtagaaaatctgatcatacttgctaacaactctcttagcagt

SEQ ID NO: 29 - protein, 19 aa, Homo sapiens
NGNVTESGCKECEELEEKN

SEQ ID NO: 30 - DNA, 57 bp, Homo sapiens
  source 1..57: mol_type = genomic DNA
aatggcaatgtcactgagtctggctgtaaagagtgtgaggaactcgaggaaaagaac

SEQ ID NO: 31 - protein, 19 aa, Homo sapiens
IKEFLQSFVHIVQMFINTS

SEQ ID NO: 32 - DNA, 57 bp, Homo sapiens
  source 1..57: mol_type = genomic DNA
ataaaggaatttcttcagtccttcgttcatatcgttcagatgtttatcaacaccagc

SEQ ID NO: 33 - protein, 127 aa, synthetic construct
APTSSSTKKTQLQLEHLLLDLQMILNGSMHIDATLYTESDVHPSCKVTAMKCFLLELQVISLESKNFHLRPRDLISNINVIVLELKGSNGNVTESGCKECEELEEKNIVEFLNRWITFCQSIISTLT

SEQ ID NO: 34 - DNA, 381 bp, synthetic construct
  source 1..381: mol_type = other DNA
gctcctacctcctccagcaccaagaaaacccagctgcagttggagcatctgctgctggacctgcagatgatcctgaacggctccatgcacatcgacgctaccctgtacaccgagtccgacgtgcacccttcctgtaaagtgaccgccatgaagtgctttctgttggagctgcaagtgatctccctggaatccaagaacttccacctgaggcctcgggacctgatctccaacatcaacgtgatcgtgctggaactgaagggctccaacggcaacgtgaccgagtctggctgtaaagagtgcgaggaactggaagagaagaacatcgtcgagtttctgaaccggtggatcaccttctgccagtccatcatctccacactgacc

SEQ ID NO: 35 - protein, 127 aa, synthetic construct
APTSSSTKKTQLQLEHLLLDLQMILNGSMHIDATLYTESDVHPSCKVTAMKCFLLELQVISLESKNFHLRPRELISNINVIVLELKGSNGNVTESGCKECEELEEKNIVEFLNRWITFCQSIISTLT

SEQ ID NO: 36 - DNA, 381 bp, synthetic construct
  source 1..381: mol_type = other DNA
gctcctacctcctccagcaccaagaaaacccagctgcagttggagcatctgctgctggacctgcagatgatcctgaacggctccatgcacatcgacgctaccctgtacaccgagtccgacgtgcacccttcctgtaaagtgaccgccatgaagtgctttctgctcgagctgcaagtgatctccctggaatccaagaacttccacctgaggccaagagagctgatctccaacatcaacgtgatcgtgctggaactgaagggctccaacggcaacgtgaccgagtctggctgtaaagagtgcgaggaactggaagagaagaacatcgtcgagtttctgaaccggtggatcaccttctgccagtccatcatctccacactgacc

SEQ ID NO: 37 - protein, 127 aa, synthetic construct
APTSSSTKKTQLQLEHLLLDLQMILNGSMHIDATLYTESDVHPSCKVTAMKCFLLELQVISLESKNFHLRPRDFISNINVIVLELKGSNGNVTESGCKECEELEEKNIVEFLNRWITFCQSIISTLT

SEQ ID NO: 38 - DNA, 381 bp, synthetic construct
  source 1..381: mol_type = other DNA
gctcctacctcctccagcaccaagaaaacccagctgcagttggagcatctgctgctggacctgcagatgatcctgaacggctccatgcacatcgacgctaccctgtacaccgagtccgacgtgcacccttcctgtaaagtgaccgccatgaagtgctttctgctcgagctgcaagtgatctccctggaatccaagaacttccacctgaggcctcgggacttcatctccaacatcaacgtgatcgtgctggaactgaagggctccaacggcaacgtgaccgagtctggctgtaaagagtgcgaggaactggaagagaagaacatcgtcgagtttctgaaccggtggatcaccttctgccagtccatcatctccacactgacc

SEQ ID NO: 39 - protein, 127 aa, synthetic construct
APTSSSTKKTQLQLEHLLLDLQMILNGSMHIDATLYTESDVHPSCKVTAMKCFLLELQVISLESKNFHLRPRDLIDNINVIVLELKGSNGNVTESGCKECEELEEKNIVEFLNRWITFCQSIISTLT

SEQ ID NO: 40 - DNA, 381 bp, synthetic construct
  source 1..381: mol_type = other DNA
gctcccacaagttcaagtactaaaaaaacccaactgcaactggagcatttgcttttggatctccaaatgattctgaatggctcaatgcacattgacgctactctttacacagagagtgatgtacacccttcttgcaaggttaccgctatgaaatgctttctcttggaactccaagtaatcagtcttgaatctaaaaattttcatttgcgcccacgcgatctgatagacaacatcaacgtgatagtactggaactcaagggaagcaatggaaacgtcacagaatcaggttgtaaagaatgtgaggaattggaagaaaagaatatagtcgagttcctcaatcgctggatcactttttgccaatccattatatccactctgaca

SEQ ID NO: 41 - protein, 127 aa, synthetic construct
APTSSSTKKTQLQLEHLLLDLQMILNGSMHIDATLYTESDVHPSCKVTAMKCFLLELQVISLESKNFHLRPRDLISDINVIVLELKGSNGNVTESGCKECEELEEKNIVEFLNRWITFCQSIISTLT

SEQ ID NO: 42 - DNA, 381 bp, synthetic construct
  source 1..381: mol_type = other DNA
gctcctacctcctccagcaccaagaaaacccagctgcagttggagcatctgctgctggacctgcagatgatcctgaacggctccatgcacatcgacgctaccctgtacaccgagtccgacgtgcacccttcctgtaaagtgaccgccatgaagtgctttctgctcgagctgcaagtgatctccctggaatccaagaacttccacctgaggcctcgggacctgatctccgacatcaacgtgatcgtgctggaactgaagggctccaacggcaacgtgaccgagtctggctgtaaagagtgcgaggaactggaagagaagaacatcgtcgagtttctgaaccggtggatcaccttctgccagtccatcatctccacactgacc

SEQ ID NO: 43 - protein, 127 aa, synthetic construct
APTSSSTKKTQLQLEHLLLDLQMILNGSMHIDATLYTESDVHPSCKVTAMKCFLLELQVISLESKNFHLRPRDLISNINLIVLELKGSNGNVTESGCKECEELEEKNIVEFLNRWITFCQSIISTLT

SEQ ID NO: 44 - DNA, 381 bp, synthetic construct
  source 1..381: mol_type = other DNA
gctcctacctcctccagcaccaagaaaacccagctgcagttggagcatctgctgctggacctgcagatgatcctgaacggctccatgcacatcgacgctaccctgtacaccgagtccgacgtgcacccttcctgtaaagtgaccgccatgaagtgctttctgctcgagctgcaagtgatctccctggaatccaagaacttccacctgaggcctcgggacctgatctccaacatcaacctgatcgtgctggaactgaagggctccaacggcaacgtgaccgagtctggctgtaaagagtgcgaggaactggaagagaagaacatcgtcgagtttctgaaccggtggatcaccttctgccagtccatcatctccacactgacc

SEQ ID NO: 45 - protein, 127 aa, synthetic construct
APTSSSTKKTQLQLEHLLLDLQMILNGSMHIDATLYTESDVHPSCKVTAMKCFLLELQVISLESKNFHLRPRDFIDDINLIVLELKGSNGNVTESGCKECEELEEKNIVEFLNRWITFCQSIISTLT

SEQ ID NO: 46 - DNA, 381 bp, synthetic construct
  source 1..381: mol_type = other DNA
gctcctacctcctccagcaccaagaaaacccagctgcagttggagcatctgctgctggacctgcagatgatcctgaacggctccatgcacatcgacgctaccctgtacaccgagtccgacgtgcacccttcctgtaaagtgaccgccatgaagtgctttctgctcgagctgcaagtgatctccctggaatccaagaacttccacctgaggcctcgggacttcatcgacgacatcaacctgatcgtgctggaactgaagggctccaacggcaacgtgaccgagtctggctgtaaagagtgcgaggaactggaagagaagaacatcgtcgagtttctgaaccggtggatcaccttctgccagtccatcatctccacactgacc

SEQ ID NO: 47 - protein, 127 aa, synthetic construct
APTSSSTKKTQLQLEHLLLDLQMILNGSMHIDATLYTESDVHPSCKVTAMKCFLLELQVISLESKNFHLRPRELIDDINLIVLELKGSNGNVTESGCKECEELEEKNIVEFLNRWITFCQSIISTLT

SEQ ID NO: 48 - DNA, 381 bp, synthetic construct
  source 1..381: mol_type = other DNA
gctcctacctcctccagcaccaagaaaacccagctgcagttggagcatctgctgctggacctgcagatgatcctgaacggctccatgcacatcgacgctaccctgtacaccgagtccgacgtgcacccttcctgtaaagtgaccgccatgaagtgctttctgctcgagctgcaagtgatctccctggaatccaagaacttccacctgaggccaagagagctgatcgacgacatcaacctgatcgtgctggaactgaagggctccaacggcaacgtgaccgagtctggctgtaaagagtgcgaggaactggaagagaagaacatcgtcgagtttctgaaccggtggatcaccttctgccagtccatcatctccacactgacc

SEQ ID NO: 49 - protein, 127 aa, synthetic construct
APTSSSTKKTQLQLEHLLLDLQMILNGSMHIDATLYTESDVHPSCKVTAMKCFLLELQVISLESKNFHLRPREFISDINLIVLELKGSNGNVTESGCKECEELEEKNIVEFLNRWITFCQSIISTLT

SEQ ID NO: 50 - DNA, 381 bp, synthetic construct
  source 1..381: mol_type = other DNA
gctcctacctcctccagcaccaagaaaacccagctgcagttggagcatctgctgctggacctgcagatgatcctgaacggctccatgcacatcgacgctaccctgtacaccgagtccgacgtgcacccttcctgtaaagtgaccgccatgaagtgctttctgctcgagctgcaagtgatctccctggaatccaagaacttccacctgaggccaagagagttcatctccgacatcaacctgatcgtgctggaactgaagggctccaacggcaacgtgaccgagtctggctgtaaagagtgcgaggaactggaagagaagaacatcgtcgagtttctgaaccggtggatcaccttctgccagtccatcatctccacactgacc

SEQ ID NO: 51 - protein, 127 aa, synthetic construct
APTSSSTKKTQLQLEHLLLDLQMILNGSMHIDATLYTESDVHPSCKVTAMKCFLLELQVISLESKNFHLRPREFIDNINLIVLELKGSNGNVTESGCKECEELEEKNIVEFLNRWITFCQSIISTLT

SEQ ID NO: 52 - DNA, 381 bp, synthetic construct
  source 1..381: mol_type = other DNA
gctcctacctcctccagcaccaagaaaacccagctgcagttggagcatctgctgctggacctgcagatgatcctgaacggctccatgcacatcgacgctaccctgtacaccgagtccgacgtgcacccttcctgtaaagtgaccgccatgaagtgctttctgctcgagctgcaagtgatctccctggaatccaagaacttccacctgaggccaagagagttcatcgacaacatcaacctgatcgtcctggaactgaagggctccaacggcaacgtgaccgagtctggctgtaaagagtgcgaggaactggaagagaagaacatcgtcgagtttctgaaccggtggatcaccttctgccagtccatcatctccacactgacc

SEQ ID NO: 53 - protein, 127 aa, synthetic construct
APTSSSTKKTQLQLEHLLLDLQMILNGSMHIDATLYTESDVHPSCKVTAMKCFLLELQVISLESKNFHLRPREFIDDINVIVLELKGSNGNVTESGCKECEELEEKNIVEFLNRWITFCQSIISTLT

SEQ ID NO: 54 - DNA, 381 bp, synthetic construct
  source 1..381: mol_type = other DNA
gctcctacctcctccagcaccaagaaaacccagctgcagttggagcatctgctgctggacctgcagatgatcctgaacggctccatgcacatcgacgctaccctgtacaccgagtccgacgtgcacccttcctgtaaagtgaccgccatgaagtgctttctgctcgagctgcaagtgatctccctggaatccaagaacttccacctgaggccaagagagttcatcgacgacatcaacgtgatcgtgctggaactgaagggctccaacggcaacgtgaccgagtctggctgtaaagagtgcgaggaactggaagagaagaacatcgtcgagtttctgaaccggtggatcaccttctgccagtccatcatctccacactgacc

SEQ ID NO: 55 - protein, 127 aa, synthetic construct
APTSSSTKKTQLQLEHLLLDLQMILNGSMHIDATLYTESDVHPSCKVTAMKCFLLELQVISLESKNFHLRPREFIDDINLIVLELKGSNGNVTESGCKECEELEEKNIVEFLNRWITFCQSIISTLT

SEQ ID NO: 56 - DNA, 381 bp, synthetic construct
  source 1..381: mol_type = other DNA
gctcctacctcctccagcaccaagaaaacccagctgcagttggagcatctgctgctggacctgcagatgatcctgaacggctccatgcacatcgacgctaccctgtacaccgagtccgacgtgcacccttcctgtaaagtgaccgccatgaagtgctttctgctcgagctgcaagtgatctccctggaatccaagaacttccacctgaggccaagagagttcatcgacgacatcaacctgatcgtgctggaactgaagggctccaacggcaacgtgaccgagtctggctgtaaagagtgcgaggaactggaagagaagaacatcgtcgagtttctgaaccggtggatcaccttctgccagtccatcatctccacactgacc

SEQ ID NO: 57 - protein, 127 aa, synthetic construct
APTSSSTKKTQLQLEHLLLDLQMILNGSMHIDATLYTESDVHPSCKVTAMKCFLLELQVISLESKNFHLRPRDLIENINVIVLELKGSNGNVTESGCKECEELEEKNIVEFLNRWITFCQSIISTLT

SEQ ID NO: 58 - DNA, 381 bp, synthetic construct
  source 1..381: mol_type = other DNA
gctcctacctcctccagcaccaagaaaacccagctgcagttggagcatctgctgctggacctgcagatgatcctgaacggctccatgcacatcgacgctaccctgtacaccgagtccgacgtgcacccttcctgtaaagtgaccgccatgaagtgctttctgttggagctgcaagtgatctccctggaatccaagaacttccacctgaggcctcgggacctgatcgaaaacatcaacgtgatcgtgctggaactgaagggctccaacggcaacgtgaccgagtctggctgtaaagagtgcgaggaactggaagagaagaacatcgtcgagtttctgaaccggtggatcaccttctgccagtccatcatctccacactgacc

SEQ ID NO: 59 - protein, 127 aa, synthetic construct
APTSSSTKKTQLQLEHLLLDLQMILNGSMHIDATLYTESDVHPSCKVTAMKCFLLELQVISLESKNFHLRPRDLINNINVIVLELKGSNGNVTESGCKECEELEEKNIVEFLNRWITFCQSIISTLT

SEQ ID NO: 60 - DNA, 381 bp, synthetic construct
  source 1..381: mol_type = other DNA
gctcctacctcctccagcaccaagaaaacccagctgcagttggagcatctgctgctggacctgcagatgatcctgaacggctccatgcacatcgacgctaccctgtacaccgagtccgacgtgcacccttcctgtaaagtgaccgccatgaagtgctttctgttggagctgcaagtgatctccctggaatccaagaacttccacctgaggcctcgggacctgatcaacaacatcaacgtgatcgtgctggaactgaagggctccaacggcaacgtgaccgagtctggctgtaaagagtgcgaggaactggaagagaagaacatcgtcgagtttctgaaccggtggatcaccttctgccagtccatcatctccacactgacc

SEQ ID NO: 61 - protein, 127 aa, synthetic construct
APTSSSTKKTQLQLEHLLLDLQMILNGSMHIDATLYTESDVHPSCKVTAMKCFLLELQVISLESKNFHLRPRDLIKNINVIVLELKGSNGNVTESGCKECEELEEKNIVEFLNRWITFCQSIISTLT

SEQ ID NO: 62 - DNA, 381 bp, synthetic construct
  source 1..381: mol_type = other DNA
gctcctacctcctccagcaccaagaaaacccagctgcagttggagcatctgctgctggacctgcagatgatcctgaacggctccatgcacatcgacgctaccctgtacaccgagtccgacgtgcacccttcctgtaaagtgaccgccatgaagtgctttctgttggagctgcaagtgatctccctggaatccaagaacttccacctgaggcctcgggacctgatcaagaacatcaacgtgatcgtgctggaactgaagggctccaacggcaacgtgaccgagtctggctgtaaagagtgcgaggaactggaagagaagaacatcgtcgagtttctgaaccggtggatcaccttctgccagtccatcatctccacactgacc

SEQ ID NO: 63 - protein, 127 aa, synthetic construct
APTSSSTKKTQLQLEHLLLDLQMILNGSMHIDATLYTESDVHPSCKVTAMKCFLLELQVISLESKNFHLRPRDLILNINVIVLELKGSNGNVTESGCKECEELEEKNIVEFLNRWITFCQSIISTLT

SEQ ID NO: 64 - DNA, 381 bp, synthetic construct
  source 1..381: mol_type = other DNA
gctcctacctcctccagcaccaagaaaacccagctgcagttggagcatctgctgctggacctgcagatgatcctgaacggctccatgcacatcgacgctaccctgtacaccgagtccgacgtgcacccttcctgtaaagtgaccgccatgaagtgctttctgttggagctgcaagtgatctccctggaatccaagaacttccacctgaggcctcgggacctgatcctcaacatcaacgtgatcgtgctggaactgaagggctccaacggcaacgtgaccgagtctggctgtaaagagtgcgaggaactggaagagaagaacatcgtcgagtttctgaaccggtggatcaccttctgccagtccatcatctccacactgacc

SEQ ID NO: 65 - protein, 127 aa, synthetic construct
APTSSSTKKTQLQLEHLLLDLQMILNGSMHIDATLYTESDVHPSCKVTAMKCFLLELQVISLESKNFHLRPRDFIDNINVIVLELKGSNGNVTESGCKECEELEEKNIVEFLNRWITFCQSIISTLT

SEQ ID NO: 66 - DNA, 381 bp, synthetic construct
  source 1..381: mol_type = other DNA
gctcctacctcctccagcaccaagaaaacccagctgcagttggagcatctgctgctggacctgcagatgatcctgaacggctccatgcacatcgacgctaccctgtacaccgagtccgacgtgcacccttcctgtaaagtgaccgccatgaagtgctttctgctcgagctgcaagtgatctccctggaatccaagaacttccacctgaggcctcgggacttcatcgacaacatcaacgtgatcgtgctggaactgaagggctccaacggcaacgtgaccgagtctggctgtaaagagtgcgaggaactggaagagaagaacatcgtcgagtttctgaaccggtggatcaccttctgccagtccatcatctccacactgacc

SEQ ID NO: 67 - protein, 127 aa, synthetic construct
APTSSSTKKTQLQLEHLLLDLQMILNGSMHIDATLYTESDVHPSCKVTAMKCFLLELQVISLESKNFHLRPRDLIDDINVIVLELKGSNGNVTESGCKECEELEEKNIVEFLNRWITFCQSIISTLT

SEQ ID NO: 68 - DNA, 381 bp, synthetic construct
  source 1..381: mol_type = other DNA
gctcctacctcctccagcaccaagaaaacccagctgcagttggagcatctgctgctggacctgcagatgatcctgaacggctccatgcacatcgacgctaccctgtacaccgagtccgacgtgcacccttcctgtaaagtgaccgccatgaagtgctttctgctcgagctgcaagtgatctccctggaatccaagaacttccacctgaggcctcgggacctgatcgacgacatcaacgtgatcgtgctggaactgaagggctccaacggcaacgtgaccgagtctggctgtaaagagtgcgaggaactggaagagaagaacatcgtcgagtttctgaaccggtggatcaccttctgccagtccatcatctccacactgacc

SEQ ID NO: 69 - protein, 127 aa, synthetic construct
APTSSSTKKTQLQLEHLLLDLQMILNGSMHIDATLYTESDVHPSCKVTAMKCFLLELQVISLESKNFHLRPRDLIDNINLIVLELKGSNGNVTESGCKECEELEEKNIVEFLNRWITFCQSIISTLT

SEQ ID NO: 70 - DNA, 381 bp, synthetic construct
  source 1..381: mol_type = other DNA
gctcctacctcctccagcaccaagaaaacccagctgcagttggagcatctgctgctggacctgcagatgatcctgaacggctccatgcacatcgacgctaccctgtacaccgagtccgacgtgcacccttcctgtaaagtgaccgccatgaagtgctttctgctcgagctgcaagtgatctccctggaatccaagaacttccacctgaggcctcgggacctgatcgacaacatcaacctgatcgtgctggaactgaagggctccaacggcaacgtgaccgagtctggctgtaaagagtgcgaggaactggaagagaagaacatcgtcgagtttctgaaccggtggatcaccttctgccagtccatcatctccacactgacc

SEQ ID NO: 71 - protein, 127 aa, synthetic construct
APTSSSTKKTQLQLEHLLLDLQMILNGSMHIDATLYTESDVHPSCKVTAMKCFLLELQVISLESKNFHLRPRDFIDDINVIVLELKGSNGNVTESGCKECEELEEKNIVEFLNRWITFCQSIISTLT

SEQ ID NO: 72 - DNA, 381 bp, synthetic construct
  source 1..381: mol_type = other DNA
gctcctacctcctccagcaccaagaaaacccagctgcagttggagcatctgctgctggacctgcagatgatcctgaacggctccatgcacatcgacgctaccctgtacaccgagtccgacgtgcacccttcctgtaaagtgaccgccatgaagtgctttctgctcgagctgcaagtgatctccctggaatccaagaacttccacctgaggcctcgggacttcatcgacgacatcaacgtgatcgtgctggaactgaagggctccaacggcaacgtgaccgagtctggctgtaaagagtgcgaggaactggaagagaagaacatcgtcgagtttctgaaccggtggatcaccttctgccagtccatcatctccacactgacc

SEQ ID NO: 73 - protein, 127 aa, synthetic construct
APTSSSTKKTQLQLEHLLLDLQMILNGSMHIDATLYTESDVHPSCKVTAMKCFLLELQVISLESKNFHLRPRDLIDDINLIVLELKGSNGNVTESGCKECEELEEKNIVEFLNRWITFCQSIISTLT

SEQ ID NO: 74 - DNA, 381 bp, synthetic construct
  source 1..381: mol_type = other DNA
gctcctacctcctccagcaccaagaaaacccagctgcagttggagcatctgctgctggacctgcagatgatcctgaacggctccatgcacatcgacgctaccctgtacaccgagtccgacgtgcacccttcctgtaaagtgaccgccatgaagtgctttctgctcgagctgcaagtgatctccctggaatccaagaacttccacctgaggcctcgggacctgatcgacgacatcaacctgatcgtgctggaactgaagggctccaacggcaacgtgaccgagtctggctgtaaagagtgcgaggaactggaagagaagaacatcgtcgagtttctgaaccggtggatcaccttctgccagtccatcatctccacactgacc

SEQ ID NO: 75 - protein, 127 aa, synthetic construct
APTSSSTKKTQLQLEHLLLDLQMILNGSMHIDATLYTESDVHPSCKVTAMKCFLLELQVISLESKNFHLRPRDFIDNINLIVLELKGSNGNVTESGCKECEELEEKNIVEFLNRWITFCQSIISTLT

SEQ ID NO: 76 - DNA, 381 bp, synthetic construct
  source 1..381: mol_type = other DNA
gctcctacctcctccagcaccaagaaaacccagctgcagttggagcatctgctgctggacctgcagatgatcctgaacggctccatgcacatcgacgctaccctgtacaccgagtccgacgtgcacccttcctgtaaagtgaccgccatgaagtgctttctgctcgagctgcaagtgatctccctggaatccaagaacttccacctgaggcctcgggacttcatcgacaacatcaacctgatcgtgctggaactgaagggctccaacggcaacgtgaccgagtctggctgtaaagagtgcgaggaactggaagagaagaacatcgtcgagtttctgaaccggtggatcaccttctgccagtccatcatctccacactgacc

SEQ ID NO: 77 - protein, 237 aa, Homo sapiens
ITCPPPMSVEHADIWVKSYSLYSRERYICNSGFKRKAGTSSLTECVLNKATNVAHWTTPSLKCIRDPALVHQRPAPPSTVTTAGVTPQPESLSPSGKEPAASSPSSNNTAATTAAIVPGSQLMPSKSPSTGTTEISSHESSHGTPSQTTAKNWELTASASHQPPGVYPQGHSDTTVAISTSTVLLCGLSAVSLLACYLKSRQTPPLASVEMEAMEALPVTWGTSSRDEDLENCSHHL

SEQ ID NO: 78 - DNA, 711 bp, Homo sapiens
  source 1..711: mol_type = genomic DNA
attacttgtccaccaccaatgtctgttgagcatgctgatatttgggtgaaatcttattctctctatagccgggaacgctatatctgcaattcaggatttaaaagaaaggctggtacctcttccttgaccgaatgtgtactgaataaagctacaaacgtggcacattggaccacgcctagccttaagtgtataagggaccccgcattagtgcatcagagacctgcacccccgagcaccgtgacaactgccggtgtcactcctcaacctgaatctctttctcccagcggtaaggaaccagctgccagtagtccgtcaagtaataataccgcagctactactgccgccatcgttcccgggtctcaactcatgccaagcaagagcccctcaaccgggacaaccgaaatttcctctcacgaaagttctcatgggactccaagccaaaccaccgctaagaattgggagttgaccgcctcagcaagtcatcaacccccaggggtatacccccaagggcattccgatactaccgttgcaattagcacttctacggtgttactttgcggattatctgcagtatccctgttggcctgttatcttaaaagccgtcagacaccgccactcgcttccgtcgagatggaagctatggaagcccttcccgtaacctggggcactagttcccgcgacgaggatctggagaattgtagtcatcatttg

SEQ ID NO: 79 - protein, 62 aa, Homo sapiens
VAISTSTVLLCGLSAVSLLACYLKSRQTPPLASVEMEAMEALPVTWGTSSRDEDLENCSHHL

SEQ ID NO: 80 - DNA, 186 bp, Homo sapiens
  source 1..186: mol_type = genomic DNA
gttgcaattagcacttctacggtgttactttgcggattatctgcagtatccctgttggcctgttatcttaaaagccgtcagacaccgccactcgcttccgtcgagatggaagctatggaagcccttcccgtaacctggggcactagttcccgcgacgaggatctggagaattgtagtcatcatttg

SEQ ID NO: 81 - protein, 65 aa, Homo sapiens
ITCPPPMSVEHADIWVKSYSLYSRERYICNSGFKRKAGTSSLTECVLNKATNVAHWTTPSLKCIR

SEQ ID NO: 82 - DNA, 195 bp, Homo sapiens
  source 1..195: mol_type = genomic DNA
attacatgccctcctccaatgtccgtggaacacgccgacatctgggtcaagtcctacagcctgtactccagagagcggtacatctgcaactccggcttcaagagaaaggccggcacctctagcctgaccgagtgcgtgctgaacaaggccaccaatgtggcccactggacaacccctagcctgaagtgtattaga

SEQ ID NO: 83 - protein, 9 aa, synthetic construct
QSFGLLDPK

SEQ ID NO: 84 - protein, 23 aa, synthetic construct
LSEGDKVKMDSRIQVLSRGVNQT

SEQ ID NO: 85 - protein, 48 aa, synthetic construct
KPTTPAPRPPTPAPTIASQPLSLRPEACRPAAGGAVHTRGLDFACDIY

SEQ ID NO: 86 - protein, 39 aa, synthetic construct
IEVMYPPPYLDNERSNGTIIHVKGKHLCPSPLFPGPSKP

SEQ ID NO: 87 - protein, 16 aa, synthetic construct
ELPTQGTFSNVSTNVS

SEQ ID NO: 88 - protein, 5 aa, synthetic construct
  REGION >5: note = The entire sequence of amino acids 1-5 can be repeated one or more times
GGGGS

SEQ ID NO: 89 - protein, 18 aa, synthetic construct
GSTGSGSKPGSGEGSTKG

SEQ ID NO: 90 - protein, 453 aa, synthetic construct
GSAESKYGPPCPPCPAPEAAGGPSVFLFPPKPKDQLMISRTPEVTCVVVDVSQEDPEVQFNWYVDGVEVHNAKTKPREEQFNSTYRVVSVLTVLHQDWLNGKEYKCKVSNKGLPSSIEKTISKAKGQPREPQVYTLPPSQEEMTKNQVSLTCLVKGFYPSDIAVEWESNGQPENNYKTTPPVLDSDGSFFLYSRLTVDKSRWQEGNVFSCSVLHEALHNHYTQKSLSLSLGGGGGSGGGGSITCPPPMSVEHADIWVKSYSLYSRERYICNSGFKRKAGTSSLTECVLNKATNVAHWTTPSLKCIRGGGGSGGGGSGGGGSGGGGSAPTSSSTKKTQLQLEHLLLDLQMILNGSMHIDATLYTESDVHPSCKVTAMKCFLLELQVISLESKNFHLRPRDLISNINVIVLELKGSNGNVTESGCKECEELEEKNIVEFLNRWITFCQSIISTLT

SEQ ID NO: 91 - protein, 453 aa, synthetic construct
GSAESKYGPPCPPCPAPEAAGGPSVFLFPPKPKDQLMISRTPEVTCVVVDVSQEDPEVQFNWYVDGVEVHNAKTKPREEQFNSTYRVVSVLTVLHQDWLNGKEYKCKVSNKGLPSSIEKTISKAKGQPREPQVYTLPPSQEEMTKNQVSLTCLVKGFYPSDIAVEWESNGQPENNYKTTPPVLDSDGSFFLYSRLTVDKSRWQEGNVFSCSVLHEALHNHYTQKSLSLSLGGGGGSGGGGSITCPPPMSVEHADIWVKSYSLYSRERYICNSGFKRKAGTSSLTECVLNKATNVAHWTTPSLKCIRGGGGSGGGGSGGGGSGGGGSAPTSSSTKKTQLQLEHLLLDLQMILNGSMHIDATLYTESDVHPSCKVTAMKCFLLELQVISLESKNFHLRPRELISNINVIVLELKGSNGNVTESGCKECEELEEKNIVEFLNRWITFCQSIISTLT

SEQ ID NO: 92 - protein, 453 aa, synthetic construct
GSAESKYGPPCPPCPAPEAAGGPSVFLFPPKPKDQLMISRTPEVTCVVVDVSQEDPEVQFNWYVDGVEVHNAKTKPREEQFNSTYRVVSVLTVLHQDWLNGKEYKCKVSNKGLPSSIEKTISKAKGQPREPQVYTLPPSQEEMTKNQVSLTCLVKGFYPSDIAVEWESNGQPENNYKTTPPVLDSDGSFFLYSRLTVDKSRWQEGNVFSCSVLHEALHNHYTQKSLSLSLGGGGGSGGGGSITCPPPMSVEHADIWVKSYSLYSRERYICNSGFKRKAGTSSLTECVLNKATNVAHWTTPSLKCIRGGGGSGGGGSGGGGSGGGGSAPTSSSTKKTQLQLEHLLLDLQMILNGSMHIDATLYTESDVHPSCKVTAMKCFLLELQVISLESKNFHLRPRDFISNINVIVLELKGSNGNVTESGCKECEELEEKNIVEFLNRWITFCQSIISTLT

SEQ ID NO: 93 - protein, 453 aa, synthetic construct
GSAESKYGPPCPPCPAPEAAGGPSVFLFPPKPKDQLMISRTPEVTCVVVDVSQEDPEVQFNWYVDGVEVHNAKTKPREEQFNSTYRVVSVLTVLHQDWLNGKEYKCKVSNKGLPSSIEKTISKAKGQPREPQVYTLPPSQEEMTKNQVSLTCLVKGFYPSDIAVEWESNGQPENNYKTTPPVLDSDGSFFLYSRLTVDKSRWQEGNVFSCSVLHEALHNHYTQKSLSLSLGGGGGSGGGGSITCPPPMSVEHADIWVKSYSLYSRERYICNSGFKRKAGTSSLTECVLNKATNVAHWTTPSLKCIRGGGGSGGGGSGGGGSGGGGSAPTSSSTKKTQLQLEHLLLDLQMILNGSMHIDATLYTESDVHPSCKVTAMKCFLLELQVISLESKNFHLRPRDLIDNINVIVLELKGSNGNVTESGCKECEELEEKNIVEFLNRWITFCQSIISTLT

SEQ ID NO: 94 - protein, 453 aa, synthetic construct
GSAESKYGPPCPPCPAPEAAGGPSVFLFPPKPKDQLMISRTPEVTCVVVDVSQEDPEVQFNWYVDGVEVHNAKTKPREEQFNSTYRVVSVLTVLHQDWLNGKEYKCKVSNKGLPSSIEKTISKAKGQPREPQVYTLPPSQEEMTKNQVSLTCLVKGFYPSDIAVEWESNGQPENNYKTTPPVLDSDGSFFLYSRLTVDKSRWQEGNVFSCSVLHEALHNHYTQKSLSLSLGGGGGSGGGGSITCPPPMSVEHADIWVKSYSLYSRERYICNSGFKRKAGTSSLTECVLNKATNVAHWTTPSLKCIRGGGGSGGGGSGGGGSGGGGSAPTSSSTKKTQLQLEHLLLDLQMILNGSMHIDATLYTESDVHPSCKVTAMKCFLLELQVISLESKNFHLRPRDLISDINVIVLELKGSNGNVTESGCKECEELEEKNIVEFLNRWITFCQSIISTLT

SEQ ID NO: 95 - protein, 453 aa, synthetic construct
GSAESKYGPPCPPCPAPEAAGGPSVFLFPPKPKDQLMISRTPEVTCVVVDVSQEDPEVQFNWYVDGVEVHNAKTKPREEQFNSTYRVVSVLTVLHQDWLNGKEYKCKVSNKGLPSSIEKTISKAKGQPREPQVYTLPPSQEEMTKNQVSLTCLVKGFYPSDIAVEWESNGQPENNYKTTPPVLDSDGSFFLYSRLTVDKSRWQEGNVFSCSVLHEALHNHYTQKSLSLSLGGGGGSGGGGSITCPPPMSVEHADIWVKSYSLYSRERYICNSGFKRKAGTSSLTECVLNKATNVAHWTTPSLKCIRGGGGSGGGGSGGGGSGGGGSAPTSSSTKKTQLQLEHLLLDLQMILNGSMHIDATLYTESDVHPSCKVTAMKCFLLELQVISLESKNFHLRPRDLISNINLIVLELKGSNGNVTESGCKECEELEEKNIVEFLNRWITFCQSIISTLT

SEQ ID NO: 96 - protein, 453 aa, synthetic construct
GSAESKYGPPCPPCPAPEAAGGPSVFLFPPKPKDQLMISRTPEVTCVVVDVSQEDPEVQFNWYVDGVEVHNAKTKPREEQFNSTYRVVSVLTVLHQDWLNGKEYKCKVSNKGLPSSIEKTISKAKGQPREPQVYTLPPSQEEMTKNQVSLTCLVKGFYPSDIAVEWESNGQPENNYKTTPPVLDSDGSFFLYSRLTVDKSRWQEGNVFSCSVLHEALHNHYTQKSLSLSLGGGGGSGGGGSITCPPPMSVEHADIWVKSYSLYSRERYICNSGFKRKAGTSSLTECVLNKATNVAHWTTPSLKCIRGGGGSGGGGSGGGGSGGGGSAPTSSSTKKTQLQLEHLLLDLQMILNGSMHIDATLYTESDVHPSCKVTAMKCFLLELQVISLESKNFHLRPRDFIDDINLIVLELKGSNGNVTESGCKECEELEEKNIVEFLNRWITFCQSIISTLT

SEQ ID NO: 97 - protein, 453 aa, synthetic construct
GSAESKYGPPCPPCPAPEAAGGPSVFLFPPKPKDQLMISRTPEVTCVVVDVSQEDPEVQFNWYVDGVEVHNAKTKPREEQFNSTYRVVSVLTVLHQDWLNGKEYKCKVSNKGLPSSIEKTISKAKGQPREPQVYTLPPSQEEMTKNQVSLTCLVKGFYPSDIAVEWESNGQPENNYKTTPPVLDSDGSFFLYSRLTVDKSRWQEGNVFSCSVLHEALHNHYTQKSLSLSLGGGGGSGGGGSITCPPPMSVEHADIWVKSYSLYSRERYICNSGFKRKAGTSSLTECVLNKATNVAHWTTPSLKCIRGGGGSGGGGSGGGGSGGGGSAPTSSSTKKTQLQLEHLLLDLQMILNGSMHIDATLYTESDVHPSCKVTAMKCFLLELQVISLESKNFHLRPRELIDDINLIVLELKGSNGNVTESGCKECEELEEKNIVEFLNRWITFCQSIISTLT

SEQ ID NO: 98 - protein, 453 aa, synthetic construct
GSAESKYGPPCPPCPAPEAAGGPSVFLFPPKPKDQLMISRTPEVTCVVVDVSQEDPEVQFNWYVDGVEVHNAKTKPREEQFNSTYRVVSVLTVLHQDWLNGKEYKCKVSNKGLPSSIEKTISKAKGQPREPQVYTLPPSQEEMTKNQVSLTCLVKGFYPSDIAVEWESNGQPENNYKTTPPVLDSDGSFFLYSRLTVDKSRWQEGNVFSCSVLHEALHNHYTQKSLSLSLGGGGGSGGGGSITCPPPMSVEHADIWVKSYSLYSRERYICNSGFKRKAGTSSLTECVLNKATNVAHWTTPSLKCIRGGGGSGGGGSGGGGSGGGGSAPTSSSTKKTQLQLEHLLLDLQMILNGSMHIDATLYTESDVHPSCKVTAMKCFLLELQVISLESKNFHLRPREFISDINLIVLELKGSNGNVTESGCKECEELEEKNIVEFLNRWITFCQSIISTLT

SEQ ID NO: 99 - protein, 453 aa, synthetic construct
GSAESKYGPPCPPCPAPEAAGGPSVFLFPPKPKDQLMISRTPEVTCVVVDVSQEDPEVQFNWYVDGVEVHNAKTKPREEQFNSTYRVVSVLTVLHQDWLNGKEYKCKVSNKGLPSSIEKTISKAKGQPREPQVYTLPPSQEEMTKNQVSLTCLVKGFYPSDIAVEWESNGQPENNYKTTPPVLDSDGSFFLYSRLTVDKSRWQEGNVFSCSVLHEALHNHYTQKSLSLSLGGGGGSGGGGSITCPPPMSVEHADIWVKSYSLYSRERYICNSGFKRKAGTSSLTECVLNKATNVAHWTTPSLKCIRGGGGSGGGGSGGGGSGGGGSAPTSSSTKKTQLQLEHLLLDLQMILNGSMHIDATLYTESDVHPSCKVTAMKCFLLELQVISLESKNFHLRPREFIDNINLIVLELKGSNGNVTESGCKECEELEEKNIVEFLNRWITFCQSIISTLT

SEQ ID NO: 100 - protein, 453 aa, synthetic construct
GSAESKYGPPCPPCPAPEAAGGPSVFLFPPKPKDQLMISRTPEVTCVVVDVSQEDPEVQFNWYVDGVEVHNAKTKPREEQFNSTYRVVSVLTVLHQDWLNGKEYKCKVSNKGLPSSIEKTISKAKGQPREPQVYTLPPSQEEMTKNQVSLTCLVKGFYPSDIAVEWESNGQPENNYKTTPPVLDSDGSFFLYSRLTVDKSRWQEGNVFSCSVLHEALHNHYTQKSLSLSLGGGGGSGGGGSITCPPPMSVEHADIWVKSYSLYSRERYICNSGFKRKAGTSSLTECVLNKATNVAHWTTPSLKCIRGGGGSGGGGSGGGGSGGGGSAPTSSSTKKTQLQLEHLLLDLQMILNGSMHIDATLYTESDVHPSCKVTAMKCFLLELQVISLESKNFHLRPREFIDNINVIVLELKGSNGNVTESGCKECEELEEKNIVEFLNRWITFCQSIISTLT

SEQ ID NO: 101 - protein, 453 aa, synthetic construct
GSAESKYGPPCPPCPAPEAAGGPSVFLFPPKPKDQLMISRTPEVTCVVVDVSQEDPEVQFNWYVDGVEVHNAKTKPREEQFNSTYRVVSVLTVLHQDWLNGKEYKCKVSNKGLPSSIEKTISKAKGQPREPQVYTLPPSQEEMTKNQVSLTCLVKGFYPSDIAVEWESNGQPENNYKTTPPVLDSDGSFFLYSRLTVDKSRWQEGNVFSCSVLHEALHNHYTQKSLSLSLGGGGGSGGGGSITCPPPMSVEHADIWVKSYSLYSRERYICNSGFKRKAGTSSLTECVLNKATNVAHWTTPSLKCIRGGGGSGGGGSGGGGSGGGGSAPTSSSTKKTQLQLEHLLLDLQMILNGSMHIDATLYTESDVHPSCKVTAMKCFLLELQVISLESKNFHLRPREFIDDINLIVLELKGSNGNVTESGCKECEELEEKNIVEFLNRWITFCQSIISTLT

SEQ ID NO: 102 - protein, 453 aa, synthetic construct
GSAESKYGPPCPPCPAPEAAGGPSVFLFPPKPKDQLMISRTPEVTCVVVDVSQEDPEVQFNWYVDGVEVHNAKTKPREEQFNSTYRVVSVLTVLHQDWLNGKEYKCKVSNKGLPSSIEKTISKAKGQPREPQVYTLPPSQEEMTKNQVSLTCLVKGFYPSDIAVEWESNGQPENNYKTTPPVLDSDGSFFLYSRLTVDKSRWQEGNVFSCSVLHEALHNHYTQKSLSLSLGGGGGSGGGGSITCPPPMSVEHADIWVKSYSLYSRERYICNSGFKRKAGTSSLTECVLNKATNVAHWTTPSLKCIRGGGGSGGGGSGGGGSGGGGSAPTSSSTKKTQLQLEHLLLDLQMILNGSMHIDATLYTESDVHPSCKVTAMKCFLLELQVISLESKNFHLRPRDLIENINVIVLELKGSNGNVTESGCKECEELEEKNIVEFLNRWITFCQSIISTLT

SEQ ID NO: 103 - protein, 453 aa, synthetic construct
GSAESKYGPPCPPCPAPEAAGGPSVFLFPPKPKDQLMISRTPEVTCVVVDVSQEDPEVQFNWYVDGVEVHNAKTKPREEQFNSTYRVVSVLTVLHQDWLNGKEYKCKVSNKGLPSSIEKTISKAKGQPREPQVYTLPPSQEEMTKNQVSLTCLVKGFYPSDIAVEWESNGQPENNYKTTPPVLDSDGSFFLYSRLTVDKSRWQEGNVFSCSVLHEALHNHYTQKSLSLSLGGGGGSGGGGSITCPPPMSVEHADIWVKSYSLYSRERYICNSGFKRKAGTSSLTECVLNKATNVAHWTTPSLKCIRGGGGSGGGGSGGGGSGGGGSAPTSSSTKKTQLQLEHLLLDLQMILNGSMHIDATLYTESDVHPSCKVTAMKCFLLELQVISLESKNFHLRPRDLINNINVIVLELKGSNGNVTESGCKECEELEEKNIVEFLNRWITFCQSIISTLT

SEQ ID NO: 104 - protein, 453 aa, synthetic construct
GSAESKYGPPCPPCPAPEAAGGPSVFLFPPKPKDQLMISRTPEVTCVVVDVSQEDPEVQFNWYVDGVEVHNAKTKPREEQFNSTYRVVSVLTVLHQDWLNGKEYKCKVSNKGLPSSIEKTISKAKGQPREPQVYTLPPSQEEMTKNQVSLTCLVKGFYPSDIAVEWESNGQPENNYKTTPPVLDSDGSFFLYSRLTVDKSRWQEGNVFSCSVLHEALHNHYTQKSLSLSLGGGGGSGGGGSITCPPPMSVEHADIWVKSYSLYSRERYICNSGFKRKAGTSSLTECVLNKATNVAHWTTPSLKCIRGGGGSGGGGSGGGGSGGGGSAPTSSSTKKTQLQLEHLLLDLQMILNGSMHIDATLYTESDVHPSCKVTAMKCFLLELQVISLESKNFHLRPRDLIKNINVIVLELKGSNGNVTESGCKECEELEEKNIVEFLNRWITFCQSIISTLT

SEQ ID NO: 105 - protein, 453 aa, synthetic construct
GSAESKYGPPCPPCPAPEAAGGPSVFLFPPKPKDQLMISRTPEVTCVVVDVSQEDPEVQFNWYVDGVEVHNAKTKPREEQFNSTYRVVSVLTVLHQDWLNGKEYKCKVSNKGLPSSIEKTISKAKGQPREPQVYTLPPSQEEMTKNQVSLTCLVKGFYPSDIAVEWESNGQPENNYKTTPPVLDSDGSFFLYSRLTVDKSRWQEGNVFSCSVLHEALHNHYTQKSLSLSLGGGGGSGGGGSITCPPPMSVEHADIWVKSYSLYSRERYICNSGFKRKAGTSSLTECVLNKATNVAHWTTPSLKCIRGGGGSGGGGSGGGGSGGGGSAPTSSSTKKTQLQLEHLLLDLQMILNGSMHIDATLYTESDVHPSCKVTAMKCFLLELQVISLESKNFHLRPRDLILNINVIVLELKGSNGNVTESGCKECEELEEKNIVEFLNRWITFCQSIISTLT

SEQ ID NO: 106 - protein, 453 aa, synthetic construct
GSAESKYGPPCPPCPAPEAAGGPSVFLFPPKPKDQLMISRTPEVTCVVVDVSQEDPEVQFNWYVDGVEVHNAKTKPREEQFNSTYRVVSVLTVLHQDWLNGKEYKCKVSNKGLPSSIEKTISKAKGQPREPQVYTLPPSQEEMTKNQVSLTCLVKGFYPSDIAVEWESNGQPENNYKTTPPVLDSDGSFFLYSRLTVDKSRWQEGNVFSCSVLHEALHNHYTQKSLSLSLGGGGGSGGGGSITCPPPMSVEHADIWVKSYSLYSRERYICNSGFKRKAGTSSLTECVLNKATNVAHWTTPSLKCIRGGGGSGGGGSGGGGSGGGGSAPTSSSTKKTQLQLEHLLLDLQMILNGSMHIDATLYTESDVHPSCKVTAMKCFLLELQVISLESKNFHLRPRDFIDNINVIVLELKGSNGNVTESGCKECEELEEKNIVEFLNRWITFCQSIISTLT

SEQ ID NO: 107 - protein, 453 aa, synthetic construct
GSAESKYGPPCPPCPAPEAAGGPSVFLFPPKPKDQLMISRTPEVTCVVVDVSQEDPEVQFNWYVDGVEVHNAKTKPREEQFNSTYRVVSVLTVLHQDWLNGKEYKCKVSNKGLPSSIEKTISKAKGQPREPQVYTLPPSQEEMTKNQVSLTCLVKGFYPSDIAVEWESNGQPENNYKTTPPVLDSDGSFFLYSRLTVDKSRWQEGNVFSCSVLHEALHNHYTQKSLSLSLGGGGGSGGGGSITCPPPMSVEHADIWVKSYSLYSRERYICNSGFKRKAGTSSLTECVLNKATNVAHWTTPSLKCIRGGGGSGGGGSGGGGSGGGGSAPTSSSTKKTQLQLEHLLLDLQMILNGSMHIDATLYTESDVHPSCKVTAMKCFLLELQVISLESKNFHLRPRDLIDDINVIVLELKGSNGNVTESGCKECEELEEKNIVEFLNRWITFCQSIISTLT

SEQ ID NO: 108 - protein, 453 aa, synthetic construct
GSAESKYGPPCPPCPAPEAAGGPSVFLFPPKPKDQLMISRTPEVTCVVVDVSQEDPEVQFNWYVDGVEVHNAKTKPREEQFNSTYRVVSVLTVLHQDWLNGKEYKCKVSNKGLPSSIEKTISKAKGQPREPQVYTLPPSQEEMTKNQVSLTCLVKGFYPSDIAVEWESNGQPENNYKTTPPVLDSDGSFFLYSRLTVDKSRWQEGNVFSCSVLHEALHNHYTQKSLSLSLGGGGGSGGGGSITCPPPMSVEHADIWVKSYSLYSRERYICNSGFKRKAGTSSLTECVLNKATNVAHWTTPSLKCIRGGGGSGGGGSGGGGSGGGGSAPTSSSTKKTQLQLEHLLLDLQMILNGSMHIDATLYTESDVHPSCKVTAMKCFLLELQVISLESKNFHLRPRDLIDNINLIVLELKGSNGNVTESGCKECEELEEKNIVEFLNRWITFCQSIISTLT

SEQ ID NO: 109 - protein, 453 aa, synthetic construct
GSAESKYGPPCPPCPAPEAAGGPSVFLFPPKPKDQLMISRTPEVTCVVVDVSQEDPEVQFNWYVDGVEVHNAKTKPREEQFNSTYRVVSVLTVLHQDWLNGKEYKCKVSNKGLPSSIEKTISKAKGQPREPQVYTLPPSQEEMTKNQVSLTCLVKGFYPSDIAVEWESNGQPENNYKTTPPVLDSDGSFFLYSRLTVDKSRWQEGNVFSCSVLHEALHNHYTQKSLSLSLGGGGGSGGGGSITCPPPMSVEHADIWVKSYSLYSRERYICNSGFKRKAGTSSLTECVLNKATNVAHWTTPSLKCIRGGGGSGGGGSGGGGSGGGGSAPTSSSTKKTQLQLEHLLLDLQMILNGSMHIDATLYTESDVHPSCKVTAMKCFLLELQVISLESKNFHLRPRDFIDDINVIVLELKGSNGNVTESGCKECEELEEKNIVEFLNRWITFCQSIISTLT

SEQ ID NO: 110 - protein, 453 aa, synthetic construct
GSAESKYGPPCPPCPAPEAAGGPSVFLFPPKPKDQLMISRTPEVTCVVVDVSQEDPEVQFNWYVDGVEVHNAKTKPREEQFNSTYRVVSVLTVLHQDWLNGKEYKCKVSNKGLPSSIEKTISKAKGQPREPQVYTLPPSQEEMTKNQVSLTCLVKGFYPSDIAVEWESNGQPENNYKTTPPVLDSDGSFFLYSRLTVDKSRWQEGNVFSCSVLHEALHNHYTQKSLSLSLGGGGGSGGGGSITCPPPMSVEHADIWVKSYSLYSRERYICNSGFKRKAGTSSLTECVLNKATNVAHWTTPSLKCIRGGGGSGGGGSGGGGSGGGGSAPTSSSTKKTQLQLEHLLLDLQMILNGSMHIDATLYTESDVHPSCKVTAMKCFLLELQVISLESKNFHLRPRDLIDDINLIVLELKGSNGNVTESGCKECEELEEKNIVEFLNRWITFCQSIISTLT

SEQ ID NO: 111 - protein, 453 aa, synthetic construct
GSAESKYGPPCPPCPAPEAAGGPSVFLFPPKPKDQLMISRTPEVTCVVVDVSQEDPEVQFNWYVDGVEVHNAKTKPREEQFNSTYRVVSVLTVLHQDWLNGKEYKCKVSNKGLPSSIEKTISKAKGQPREPQVYTLPPSQEEMTKNQVSLTCLVKGFYPSDIAVEWESNGQPENNYKTTPPVLDSDGSFFLYSRLTVDKSRWQEGNVFSCSVLHEALHNHYTQKSLSLSLGGGGGSGGGGSITCPPPMSVEHADIWVKSYSLYSRERYICNSGFKRKAGTSSLTECVLNKATNVAHWTTPSLKCIRGGGGSGGGGSGGGGSGGGGSAPTSSSTKKTQLQLEHLLLDLQMILNGSMHIDATLYTESDVHPSCKVTAMKCFLLELQVISLESKNFHLRPRDFIDNINLIVLELKGSNGNVTESGCKECEELEEKNIVEFLNRWITFCQSIISTLT

SEQ ID NO: 112 - protein, 453 aa, synthetic construct
APTSSSTKKTQLQLEHLLLDLQMILNGSMHIDATLYTESDVHPSCKVTAMKCFLLELQVISLESKNFHLRPRDLISNINVIVLELKGSNGNVTESGCKECEELEEKNIVEFLNRWITFCQSIISTLTGGGGSGGGGSGGGGSGGGGSITCPPPMSVEHADIWVKSYSLYSRERYICNSGFKRKAGTSSLTECVLNKATNVAHWTTPSLKCIRGGGGSGGGGSGSAESKYGPPCPPCPAPEAAGGPSVFLFPPKPKDQLMISRTPEVTCVVVDVSQEDPEVQFNWYVDGVEVHNAKTKPREEQFNSTYRVVSVLTVLHQDWLNGKEYKCKVSNKGLPSSIEKTISKAKGQPREPQVYTLPPSQEEMTKNQVSLTCLVKGFYPSDIAVEWESNGQPENNYKTTPPVLDSDGSFFLYSRLTVDKSRWQEGNVFSCSVLHEALHNHYTQKSLSLSLG

SEQ ID NO: 113 - protein, 453 aa, synthetic construct
APTSSSTKKTQLQLEHLLLDLQMILNGSMHIDATLYTESDVHPSCKVTAMKCFLLELQVISLESKNFHLRPRELISNINVIVLELKGSNGNVTESGCKECEELEEKNIVEFLNRWITFCQSIISTLTGGGGSGGGGSGGGGSGGGGSITCPPPMSVEHADIWVKSYSLYSRERYICNSGFKRKAGTSSLTECVLNKATNVAHWTTPSLKCIRGGGGSGGGGSGSAESKYGPPCPPCPAPEAAGGPSVFLFPPKPKDQLMISRTPEVTCVVVDVSQEDPEVQFNWYVDGVEVHNAKTKPREEQFNSTYRVVSVLTVLHQDWLNGKEYKCKVSNKGLPSSIEKTISKAKGQPREPQVYTLPPSQEEMTKNQVSLTCLVKGFYPSDIAVEWESNGQPENNYKTTPPVLDSDGSFFLYSRLTVDKSRWQEGNVFSCSVLHEALHNHYTQKSLSLSLG

SEQ ID NO: 114 - protein, 453 aa, synthetic construct
APTSSSTKKTQLQLEHLLLDLQMILNGSMHIDATLYTESDVHPSCKVTAMKCFLLELQVISLESKNFHLRPRDFISNINVIVLELKGSNGNVTESGCKECEELEEKNIVEFLNRWITFCQSIISTLTGGGGSGGGGSGGGGSGGGGSITCPPPMSVEHADIWVKSYSLYSRERYICNSGFKRKAGTSSLTECVLNKATNVAHWTTPSLKCIRGGGGSGGGGSGSAESKYGPPCPPCPAPEAAGGPSVFLFPPKPKDQLMISRTPEVTCVVVDVSQEDPEVQFNWYVDGVEVHNAKTKPREEQFNSTYRVVSVLTVLHQDWLNGKEYKCKVSNKGLPSSIEKTISKAKGQPREPQVYTLPPSQEEMTKNQVSLTCLVKGFYPSDIAVEWESNGQPENNYKTTPPVLDSDGSFFLYSRLTVDKSRWQEGNVFSCSVLHEALHNHYTQKSLSLSLG

SEQ ID NO: 115 - protein, 453 aa, synthetic construct
APTSSSTKKTQLQLEHLLLDLQMILNGSMHIDATLYTESDVHPSCKVTAMKCFLLELQVISLESKNFHLRPRDLIDNINVIVLELKGSNGNVTESGCKECEELEEKNIVEFLNRWITFCQSIISTLTGGGGSGGGGSGGGGSGGGGSITCPPPMSVEHADIWVKSYSLYSRERYICNSGFKRKAGTSSLTECVLNKATNVAHWTTPSLKCIRGGGGSGGGGSGSAESKYGPPCPPCPAPEAAGGPSVFLFPPKPKDQLMISRTPEVTCVVVDVSQEDPEVQFNWYVDGVEVHNAKTKPREEQFNSTYRVVSVLTVLHQDWLNGKEYKCKVSNKGLPSSIEKTISKAKGQPREPQVYTLPPSQEEMTKNQVSLTCLVKGFYPSDIAVEWESNGQPENNYKTTPPVLDSDGSFFLYSRLTVDKSRWQEGNVFSCSVLHEALHNHYTQKSLSLSLG

SEQ ID NO: 116 - protein, 453 aa, synthetic construct
APTSSSTKKTQLQLEHLLLDLQMILNGSMHIDATLYTESDVHPSCKVTAMKCFLLELQVISLESKNFHLRPRDLISDINVIVLELKGSNGNVTESGCKECEELEEKNIVEFLNRWITFCQSIISTLTGGGGSGGGGSGGGGSGGGGSITCPPPMSVEHADIWVKSYSLYSRERYICNSGFKRKAGTSSLTECVLNKATNVAHWTTPSLKCIRGGGGSGGGGSGSAESKYGPPCPPCPAPEAAGGPSVFLFPPKPKDQLMISRTPEVTCVVVDVSQEDPEVQFNWYVDGVEVHNAKTKPREEQFNSTYRVVSVLTVLHQDWLNGKEYKCKVSNKGLPSSIEKTISKAKGQPREPQVYTLPPSQEEMTKNQVSLTCLVKGFYPSDIAVEWESNGQPENNYKTTPPVLDSDGSFFLYSRLTVDKSRWQEGNVFSCSVLHEALHNHYTQKSLSLSLG

SEQ ID NO: 117 - protein, 453 aa, synthetic construct
APTSSSTKKTQLQLEHLLLDLQMILNGSMHIDATLYTESDVHPSCKVTAMKCFLLELQVISLESKNFHLRPRDLISNINLIVLELKGSNGNVTESGCKECEELEEKNIVEFLNRWITFCQSIISTLTGGGGSGGGGSGGGGSGGGGSITCPPPMSVEHADIWVKSYSLYSRERYICNSGFKRKAGTSSLTECVLNKATNVAHWTTPSLKCIRGGGGSGGGGSGSAESKYGPPCPPCPAPEAAGGPSVFLFPPKPKDQLMISRTPEVTCVVVDVSQEDPEVQFNWYVDGVEVHNAKTKPREEQFNSTYRVVSVLTVLHQDWLNGKEYKCKVSNKGLPSSIEKTISKAKGQPREPQVYTLPPSQEEMTKNQVSLTCLVKGFYPSDIAVEWESNGQPENNYKTTPPVLDSDGSFFLYSRLTVDKSRWQEGNVFSCSVLHEALHNHYTQKSLSLSLG

SEQ ID NO: 118 - protein, 453 aa, synthetic construct
APTSSSTKKTQLQLEHLLLDLQMILNGSMHIDATLYTESDVHPSCKVTAMKCFLLELQVISLESKNFHLRPRDFIDDINLIVLELKGSNGNVTESGCKECEELEEKNIVEFLNRWITFCQSIISTLTGGGGSGGGGSGGGGSGGGGSITCPPPMSVEHADIWVKSYSLYSRERYICNSGFKRKAGTSSLTECVLNKATNVAHWTTPSLKCIRGGGGSGGGGSGSAESKYGPPCPPCPAPEAAGGPSVFLFPPKPKDQLMISRTPEVTCVVVDVSQEDPEVQFNWYVDGVEVHNAKTKPREEQFNSTYRVVSVLTVLHQDWLNGKEYKCKVSNKGLPSSIEKTISKAKGQPREPQVYTLPPSQEEMTKNQVSLTCLVKGFYPSDIAVEWESNGQPENNYKTTPPVLDSDGSFFLYSRLTVDKSRWQEGNVFSCSVLHEALHNHYTQKSLSLSLG

SEQ ID NO: 119 - protein, 453 aa, synthetic construct
APTSSSTKKTQLQLEHLLLDLQMILNGSMHIDATLYTESDVHPSCKVTAMKCFLLELQVISLESKNFHLRPRELIDDINLIVLELKGSNGNVTESGCKECEELEEKNIVEFLNRWITFCQSIISTLTGGGGSGGGGSGGGGSGGGGSITCPPPMSVEHADIWVKSYSLYSRERYICNSGFKRKAGTSSLTECVLNKATNVAHWTTPSLKCIRGGGGSGGGGSGSAESKYGPPCPPCPAPEAAGGPSVFLFPPKPKDQLMISRTPEVTCVVVDVSQEDPEVQFNWYVDGVEVHNAKTKPREEQFNSTYRVVSVLTVLHQDWLNGKEYKCKVSNKGLPSSIEKTISKAKGQPREPQVYTLPPSQEEMTKNQVSLTCLVKGFYPSDIAVEWESNGQPENNYKTTPPVLDSDGSFFLYSRLTVDKSRWQEGNVFSCSVLHEALHNHYTQKSLSLSLG

SEQ ID NO: 120 - protein, 453 aa, synthetic construct
APTSSSTKKTQLQLEHLLLDLQMILNGSMHIDATLYTESDVHPSCKVTAMKCFLLELQVISLESKNFHLRPREFISDINLIVLELKGSNGNVTESGCKECEELEEKNIVEFLNRWITFCQSIISTLTGGGGSGGGGSGGGGSGGGGSITCPPPMSVEHADIWVKSYSLYSRERYICNSGFKRKAGTSSLTECVLNKATNVAHWTTPSLKCIRGGGGSGGGGSGSAESKYGPPCPPCPAPEAAGGPSVFLFPPKPKDQLMISRTPEVTCVVVDVSQEDPEVQFNWYVDGVEVHNAKTKPREEQFNSTYRVVSVLTVLHQDWLNGKEYKCKVSNKGLPSSIEKTISKAKGQPREPQVYTLPPSQEEMTKNQVSLTCLVKGFYPSDIAVEWESNGQPENNYKTTPPVLDSDGSFFLYSRLTVDKSRWQEGNVFSCSVLHEALHNHYTQKSLSLSLG

SEQ ID NO: 121 - protein, 453 aa, synthetic construct
APTSSSTKKTQLQLEHLLLDLQMILNGSMHIDATLYTESDVHPSCKVTAMKCFLLELQVISLESKNFHLRPREFIDNINLIVLELKGSNGNVTESGCKECEELEEKNIVEFLNRWITFCQSIISTLTGGGGSGGGGSGGGGSGGGGSITCPPPMSVEHADIWVKSYSLYSRERYICNSGFKRKAGTSSLTECVLNKATNVAHWTTPSLKCIRGGGGSGGGGSGSAESKYGPPCPPCPAPEAAGGPSVFLFPPKPKDQLMISRTPEVTCVVVDVSQEDPEVQFNWYVDGVEVHNAKTKPREEQFNSTYRVVSVLTVLHQDWLNGKEYKCKVSNKGLPSSIEKTISKAKGQPREPQVYTLPPSQEEMTKNQVSLTCLVKGFYPSDIAVEWESNGQPENNYKTTPPVLDSDGSFFLYSRLTVDKSRWQEGNVFSCSVLHEALHNHYTQKSLSLSLG

SEQ ID NO: 122 - protein, 453 aa, synthetic construct
APTSSSTKKTQLQLEHLLLDLQMILNGSMHIDATLYTESDVHPSCKVTAMKCFLLELQVISLESKNFHLRPREFIDDINVIVLELKGSNGNVTESGCKECEELEEKNIVEFLNRWITFCQSIISTLTGGGGSGGGGSGGGGSGGGGSITCPPPMSVEHADIWVKSYSLYSRERYICNSGFKRKAGTSSLTECVLNKATNVAHWTTPSLKCIRGGGGSGGGGSGSAESKYGPPCPPCPAPEAAGGPSVFLFPPKPKDQLMISRTPEVTCVVVDVSQEDPEVQFNWYVDGVEVHNAKTKPREEQFNSTYRVVSVLTVLHQDWLNGKEYKCKVSNKGLPSSIEKTISKAKGQPREPQVYTLPPSQEEMTKNQVSLTCLVKGFYPSDIAVEWESNGQPENNYKTTPPVLDSDGSFFLYSRLTVDKSRWQEGNVFSCSVLHEALHNHYTQKSLSLSLG

SEQ ID NO: 123 - protein, 453 aa, synthetic construct
APTSSSTKKTQLQLEHLLLDLQMILNGSMHIDATLYTESDVHPSCKVTAMKCFLLELQVISLESKNFHLRPREFIDDINLIVLELKGSNGNVTESGCKECEELEEKNIVEFLNRWITFCQSIISTLTGGGGSGGGGSGGGGSGGGGSITCPPPMSVEHADIWVKSYSLYSRERYICNSGFKRKAGTSSLTECVLNKATNVAHWTTPSLKCIRGGGGSGGGGSGSAESKYGPPCPPCPAPEAAGGPSVFLFPPKPKDQLMISRTPEVTCVVVDVSQEDPEVQFNWYVDGVEVHNAKTKPREEQFNSTYRVVSVLTVLHQDWLNGKEYKCKVSNKGLPSSIEKTISKAKGQPREPQVYTLPPSQEEMTKNQVSLTCLVKGFYPSDIAVEWESNGQPENNYKTTPPVLDSDGSFFLYSRLTVDKSRWQEGNVFSCSVLHEALHNHYTQKSLSLSLG

SEQ ID NO: 124 - protein, 453 aa, synthetic construct
APTSSSTKKTQLQLEHLLLDLQMILNGSMHIDATLYTESDVHPSCKVTAMKCFLLELQVISLESKNFHLRPRDLIENINVIVLELKGSNGNVTESGCKECEELEEKNIVEFLNRWITFCQSIISTLTGGGGSGGGGSGGGGSGGGGSITCPPPMSVEHADIWVKSYSLYSRERYICNSGFKRKAGTSSLTECVLNKATNVAHWTTPSLKCIRGGGGSGGGGSGSAESKYGPPCPPCPAPEAAGGPSVFLFPPKPKDQLMISRTPEVTCVVVDVSQEDPEVQFNWYVDGVEVHNAKTKPREEQFNSTYRVVSVLTVLHQDWLNGKEYKCKVSNKGLPSSIEKTISKAKGQPREPQVYTLPPSQEEMTKNQVSLTCLVKGFYPSDIAVEWESNGQPENNYKTTPPVLDSDGSFFLYSRLTVDKSRWQEGNVFSCSVLHEALHNHYTQKSLSLSLG

SEQ ID NO: 125 - protein, 453 aa, synthetic construct
APTSSSTKKTQLQLEHLLLDLQMILNGSMHIDATLYTESDVHPSCKVTAMKCFLLELQVISLESKNFHLRPRDLINNINVIVLELKGSNGNVTESGCKECEELEEKNIVEFLNRWITFCQSIISTLTGGGGSGGGGSGGGGSGGGGSITCPPPMSVEHADIWVKSYSLYSRERYICNSGFKRKAGTSSLTECVLNKATNVAHWTTPSLKCIRGGGGSGGGGSGSAESKYGPPCPPCPAPEAAGGPSVFLFPPKPKDQLMISRTPEVTCVVVDVSQEDPEVQFNWYVDGVEVHNAKTKPREEQFNSTYRVVSVLTVLHQDWLNGKEYKCKVSNKGLPSSIEKTISKAKGQPREPQVYTLPPSQEEMTKNQVSLTCLVKGFYPSDIAVEWESNGQPENNYKTTPPVLDSDGSFFLYSRLTVDKSRWQEGNVFSCSVLHEALHNHYTQKSLSLSLG

SEQ ID NO: 126 - protein, 453 aa, synthetic construct
APTSSSTKKTQLQLEHLLLDLQMILNGSMHIDATLYTESDVHPSCKVTAMKCFLLELQVISLESKNFHLRPRDLIKNINVIVLELKGSNGNVTESGCKECEELEEKNIVEFLNRWITFCQSIISTLTGGGGSGGGGSGGGGSGGGGSITCPPPMSVEHADIWVKSYSLYSRERYICNSGFKRKAGTSSLTECVLNKATNVAHWTTPSLKCIRGGGGSGGGGSGSAESKYGPPCPPCPAPEAAGGPSVFLFPPKPKDQLMISRTPEVTCVVVDVSQEDPEVQFNWYVDGVEVHNAKTKPREEQFNSTYRVVSVLTVLHQDWLNGKEYKCKVSNKGLPSSIEKTISKAKGQPREPQVYTLPPSQEEMTKNQVSLTCLVKGFYPSDIAVEWESNGQPENNYKTTPPVLDSDGSFFLYSRLTVDKSRWQEGNVFSCSVLHEALHNHYTQKSLSLSLG

SEQ ID NO: 127 - protein, 453 aa, synthetic construct
APTSSSTKKTQLQLEHLLLDLQMILNGSMHIDATLYTESDVHPSCKVTAMKCFLLELQVISLESKNFHLRPRDLILNINVIVLELKGSNGNVTESGCKECEELEEKNIVEFLNRWITFCQSIISTLTGGGGSGGGGSGGGGSGGGGSITCPPPMSVEHADIWVKSYSLYSRERYICNSGFKRKAGTSSLTECVLNKATNVAHWTTPSLKCIRGGGGSGGGGSGSAESKYGPPCPPCPAPEAAGGPSVFLFPPKPKDQLMISRTPEVTCVVVDVSQEDPEVQFNWYVDGVEVHNAKTKPREEQFNSTYRVVSVLTVLHQDWLNGKEYKCKVSNKGLPSSIEKTISKAKGQPREPQVYTLPPSQEEMTKNQVSLTCLVKGFYPSDIAVEWESNGQPENNYKTTPPVLDSDGSFFLYSRLTVDKSRWQEGNVFSCSVLHEALHNHYTQKSLSLSLG

SEQ ID NO: 128 - protein, 453 aa, synthetic construct
APTSSSTKKTQLQLEHLLLDLQMILNGSMHIDATLYTESDVHPSCKVTAMKCFLLELQVISLESKNFHLRPRDFIDNINVIVLELKGSNGNVTESGCKECEELEEKNIVEFLNRWITFCQSIISTLTGGGGSGGGGSGGGGSGGGGSITCPPPMSVEHADIWVKSYSLYSRERYICNSGFKRKAGTSSLTECVLNKATNVAHWTTPSLKCIRGGGGSGGGGSGSAESKYGPPCPPCPAPEAAGGPSVFLFPPKPKDQLMISRTPEVTCVVVDVSQEDPEVQFNWYVDGVEVHNAKTKPREEQFNSTYRVVSVLTVLHQDWLNGKEYKCKVSNKGLPSSIEKTISKAKGQPREPQVYTLPPSQEEMTKNQVSLTCLVKGFYPSDIAVEWESNGQPENNYKTTPPVLDSDGSFFLYSRLTVDKSRWQEGNVFSCSVLHEALHNHYTQKSLSLSLG

SEQ ID NO: 129 - protein, 453 aa, synthetic construct
APTSSSTKKTQLQLEHLLLDLQMILNGSMHIDATLYTESDVHPSCKVTAMKCFLLELQVISLESKNFHLRPRDLIDDINVIVLELKGSNGNVTESGCKECEELEEKNIVEFLNRWITFCQSIISTLTGGGGSGGGGSGGGGSGGGGSITCPPPMSVEHADIWVKSYSLYSRERYICNSGFKRKAGTSSLTECVLNKATNVAHWTTPSLKCIRGGGGSGGGGSGSAESKYGPPCPPCPAPEAAGGPSVFLFPPKPKDQLMISRTPEVTCVVVDVSQEDPEVQFNWYVDGVEVHNAKTKPREEQFNSTYRVVSVLTVLHQDWLNGKEYKCKVSNKGLPSSIEKTISKAKGQPREPQVYTLPPSQEEMTKNQVSLTCLVKGFYPSDIAVEWESNGQPENNYKTTPPVLDSDGSFFLYSRLTVDKSRWQEGNVFSCSVLHEALHNHYTQKSLSLSLG

SEQ ID NO: 130 - protein, 453 aa, synthetic construct
APTSSSTKKTQLQLEHLLLDLQMILNGSMHIDATLYTESDVHPSCKVTAMKCFLLELQVISLESKNFHLRPRDLIDNINLIVLELKGSNGNVTESGCKECEELEEKNIVEFLNRWITFCQSIISTLTGGGGSGGGGSGGGGSGGGGSITCPPPMSVEHADIWVKSYSLYSRERYICNSGFKRKAGTSSLTECVLNKATNVAHWTTPSLKCIRGGGGSGGGGSGSAESKYGPPCPPCPAPEAAGGPSVFLFPPKPKDQLMISRTPEVTCVVVDVSQEDPEVQFNWYVDGVEVHNAKTKPREEQFNSTYRVVSVLTVLHQDWLNGKEYKCKVSNKGLPSSIEKTISKAKGQPREPQVYTLPPSQEEMTKNQVSLTCLVKGFYPSDIAVEWESNGQPENNYKTTPPVLDSDGSFFLYSRLTVDKSRWQEGNVFSCSVLHEALHNHYTQKSLSLSLG

SEQ ID NO: 131 - protein, 453 aa, synthetic construct
APTSSSTKKTQLQLEHLLLDLQMILNGSMHIDATLYTESDVHPSCKVTAMKCFLLELQVISLESKNFHLRPRDFIDDINVIVLELKGSNGNVTESGCKECEELEEKNIVEFLNRWITFCQSIISTLTGGGGSGGGGSGGGGSGGGGSITCPPPMSVEHADIWVKSYSLYSRERYICNSGFKRKAGTSSLTECVLNKATNVAHWTTPSLKCIRGGGGSGGGGSGSAESKYGPPCPPCPAPEAAGGPSVFLFPPKPKDQLMISRTPEVTCVVVDVSQEDPEVQFNWYVDGVEVHNAKTKPREEQFNSTYRVVSVLTVLHQDWLNGKEYKCKVSNKGLPSSIEKTISKAKGQPREPQVYTLPPSQEEMTKNQVSLTCLVKGFYPSDIAVEWESNGQPENNYKTTPPVLDSDGSFFLYSRLTVDKSRWQEGNVFSCSVLHEALHNHYTQKSLSLSLG

SEQ ID NO: 132 - protein, 453 aa, synthetic construct
APTSSSTKKTQLQLEHLLLDLQMILNGSMHIDATLYTESDVHPSCKVTAMKCFLLELQVISLESKNFHLRPRDLIDDINLIVLELKGSNGNVTESGCKECEELEEKNIVEFLNRWITFCQSIISTLTGGGGSGGGGSGGGGSGGGGSITCPPPMSVEHADIWVKSYSLYSRERYICNSGFKRKAGTSSLTECVLNKATNVAHWTTPSLKCIRGGGGSGGGGSGSAESKYGPPCPPCPAPEAAGGPSVFLFPPKPKDQLMISRTPEVTCVVVDVSQEDPEVQFNWYVDGVEVHNAKTKPREEQFNSTYRVVSVLTVLHQDWLNGKEYKCKVSNKGLPSSIEKTISKAKGQPREPQVYTLPPSQEEMTKNQVSLTCLVKGFYPSDIAVEWESNGQPENNYKTTPPVLDSDGSFFLYSRLTVDKSRWQEGNVFSCSVLHEALHNHYTQKSLSLSLG

SEQ ID NO: 133 - protein, 453 aa, synthetic construct
APTSSSTKKTQLQLEHLLLDLQMILNGSMHIDATLYTESDVHPSCKVTAMKCFLLELQVISLESKNFHLRPRDFIDNINLIVLELKGSNGNVTESGCKECEELEEKNIVEFLNRWITFCQSIISTLTGGGGSGGGGSGGGGSGGGGSITCPPPMSVEHADIWVKSYSLYSRERYICNSGFKRKAGTSSLTECVLNKATNVAHWTTPSLKCIRGGGGSGGGGSGSAESKYGPPCPPCPAPEAAGGPSVFLFPPKPKDQLMISRTPEVTCVVVDVSQEDPEVQFNWYVDGVEVHNAKTKPREEQFNSTYRVVSVLTVLHQDWLNGKEYKCKVSNKGLPSSIEKTISKAKGQPREPQVYTLPPSQEEMTKNQVSLTCLVKGFYPSDIAVEWESNGQPENNYKTTPPVLDSDGSFFLYSRLTVDKSRWQEGNVFSCSVLHEALHNHYTQKSLSLSLG

SEQ ID NO: 134 - protein, 367 aa, synthetic construct
AESKYGPPCPPCPAPEAAGGPSVFLFPPKPKDTLMISRTPEVTCVVVDVSQEDPEVQFNWYVDGVEVHNAKTKPREEQFNSTYRVVSVLTVLHQDWLNGKEYKCKVSNKGLPSSIEKTISKAKGQPREPQVYTLPPSQEEMTKNQVSLTCLVKGFYPSDIAVEWESNGQPENNYKTTPPVLDSDGSFFLYSRLTVDKSRWQEGNVFSCSVMHEALHNHYTQKSLSLSLGGGGGSAPTSSSTKKTQLQLEHLLLDLQMILNGINNYKNPKLTRMLTFKFYMPKKATELKHLQCLEEELKPLEEVLNLAQSKNFHLRPRDLISNINVIVLELKGSETTFMCEYADETATIVEFLNRWITFCQSIISTLT

SEQ ID NO: 135 - DNA, 1359 bp, synthetic construct
  source 1..1359: mol_type = other DNA
ggatccgccgagtctaagtacggccctccttgtcctccatgtcctgctccagaagctgccggagggcccagtgtgtttctgttccctccaaagcctaaggaccagctgatgatctctcggacccctgaagtgacctgcgtggtggtggatgtgtcccaagaggaccctgaggtgcagttcaattggtacgtggacggcgtggaagtgcacaacgccaagaccaagcctagagaggaacagttcaactccacctacagagtggtgtccgtgctgaccgtgctgcaccaggattggctgaacggcaaagagtacaagtgcaaggtgtccaacaagggcctgccttccagcatcgaaaagaccatctccaaggccaagggccagcctagggaaccccaggtttacaccctgcctccaagccaagaggaaatgaccaagaaccaggtgtccctgacctgcctggtcaagggcttctacccttccgatatcgccgtggaatgggagagcaatggccagcctgagaacaactacaagaccacacctcctgtgctggactccgacggctccttctttctgtactcccgcctgaccgtggacaagtccagatggcaagagggcaacgtgttctcctgctctgtgctgcacgaggccctgcacaatcactacacccagaagtccctgtctctgtcccttggcggtggcggaggatctggcggaggcggatctattacatgccctcctccaatgtccgtggaacacgccgacatctgggtcaagtcctacagcctgtactccagagagcggtacatctgcaactccggcttcaagagaaaggccggcacctctagcctgaccgagtgcgtgctgaacaaggccaccaatgtggcccactggacaacccctagcctgaagtgtattagaggcggcggaggaagcggtggcggcggtagcggaggtggtggttctggtggtggcggttctgctcctacctcctccagcaccaagaaaacccagctgcagttggagcatctgctgctggacctgcagatgatcctgaacggctccatgcacatcgacgctaccctgtacaccgagtccgacgtgcacccttcctgtaaagtgaccgccatgaagtgctttctgttggagctgcaagtgatctccctggaatccaagaacttccacctgaggcctcgggacctgatctccaacatcaacgtgatcgtgctggaactgaagggctccaacggcaacgtgaccgagtctggctgtaaagagtgcgaggaactggaagagaagaacatcgtcgagtttctgaaccggtggatcaccttctgccagtccatcatctccacactgacc

SEQ ID NO: 136 - DNA, 1359 bp, synthetic construct
  source 1..1359: mol_type = other DNA
ggatccgccgagtctaagtacggccctccttgtcctccatgtcctgctccagaagctgccggagggcccagtgtgtttctgttccctccaaagcctaaggaccagctgatgatctctcggacccctgaagtgacctgcgtggtggtggatgtgtcccaagaggaccctgaggtgcagttcaattggtacgtggacggcgtggaagtgcacaacgccaagaccaagcctagagaggaacagttcaactccacctacagagtggtgtccgtgctgaccgtgctgcaccaggattggctgaacggcaaagagtacaagtgcaaggtgtccaacaagggcctgccttccagcatcgaaaagaccatctccaaggccaagggccagcctagggaaccccaggtttacaccctgcctccaagccaagaggaaatgaccaagaaccaggtgtccctgacctgcctggtcaagggcttctacccttccgatatcgccgtggaatgggagagcaatggccagcctgagaacaactacaagaccacacctcctgtgctggactccgacggctccttctttctgtactcccgcctgaccgtggacaagtccagatggcaagagggcaacgtgttctcctgctctgtgctgcacgaggccctgcacaatcactacacccagaagtccctgtctctgtcccttggcggtggcggaggatctggcggaggcggatctattacatgccctcctccaatgtccgtggaacacgccgacatctgggtcaagtcctacagcctgtactccagagagcggtacatctgcaactccggcttcaagagaaaggccggcacctctagcctgaccgagtgcgtgctgaacaaggccaccaatgtggcccactggacaacccctagcctgaagtgtattagaggcggcggaggaagcggtggcggcggtagcggaggtggtggttctggtggtggcggttctgctcctacctcctccagcaccaagaaaacccagctgcagttggagcatctgctgctggacctgcagatgatcctgaacggctccatgcacatcgacgctaccctgtacaccgagtccgacgtgcacccttcctgtaaagtgaccgccatgaagtgctttctgctcgagctgcaagtgatctccctggaatccaagaacttccacctgaggccaagagagctgatctccaacatcaacgtgatcgtgctggaactgaagggctccaacggcaacgtgaccgagtctggctgtaaagagtgcgaggaactggaagagaagaacatcgtcgagtttctgaaccggtggatcaccttctgccagtccatcatctccacactgacc

SEQ ID NO: 137 - DNA, 1359 bp, synthetic construct
  source 1..1359: mol_type = other DNA
ggatccgccgagtctaagtacggccctccttgtcctccatgtcctgctccagaagctgccggagggcccagtgtgtttctgttccctccaaagcctaaggaccagctgatgatctctcggacccctgaagtgacctgcgtggtggtggatgtgtcccaagaggaccctgaggtgcagttcaattggtacgtggacggcgtggaagtgcacaacgccaagaccaagcctagagaggaacagttcaactccacctacagagtggtgtccgtgctgaccgtgctgcaccaggattggctgaacggcaaagagtacaagtgcaaggtgtccaacaagggcctgccttccagcatcgaaaagaccatctccaaggccaagggccagcctagggaaccccaggtttacaccctgcctccaagccaagaggaaatgaccaagaaccaggtgtccctgacctgcctggtcaagggcttctacccttccgatatcgccgtggaatgggagagcaatggccagcctgagaacaactacaagaccacacctcctgtgctggactccgacggctccttctttctgtactcccgcctgaccgtggacaagtccagatggcaagagggcaacgtgttctcctgctctgtgctgcacgaggccctgcacaatcactacacccagaagtccctgtctctgtcccttggcggtggcggaggatctggcggaggcggatctattacatgccctcctccaatgtccgtggaacacgccgacatctgggtcaagtcctacagcctgtactccagagagcggtacatctgcaactccggcttcaagagaaaggccggcacctctagcctgaccgagtgcgtgctgaacaaggccaccaatgtggcccactggacaacccctagcctgaagtgtattagaggcggcggaggaagcggtggcggcggtagcggaggtggtggttctggtggtggcggttctgctcctacctcctccagcaccaagaaaacccagctgcagttggagcatctgctgctggacctgcagatgatcctgaacggctccatgcacatcgacgctaccctgtacaccgagtccgacgtgcacccttcctgtaaagtgaccgccatgaagtgctttctgctcgagctgcaagtgatctccctggaatccaagaacttccacctgaggcctcgggacttcatctccaacatcaacgtgatcgtgctggaactgaagggctccaacggcaacgtgaccgagtctggctgtaaagagtgcgaggaactggaagagaagaacatcgtcgagtttctgaaccggtggatcaccttctgccagtccatcatctccacactgacc

SEQ ID NO: 138 - DNA, 1359 bp, synthetic construct
  source 1..1359: mol_type = other DNA
ggatccgccgagtctaagtacggccctccttgtcctccatgtcctgctccagaagctgccggagggcccagtgtgtttctgttccctccaaagcctaaggaccagctgatgatctctcggacccctgaagtgacctgcgtggtggtggatgtgtcccaagaggaccctgaggtgcagttcaattggtacgtggacggcgtggaagtgcacaacgccaagaccaagcctagagaggaacagttcaactccacctacagagtggtgtccgtgctgaccgtgctgcaccaggattggctgaacggcaaagagtacaagtgcaaggtgtccaacaagggcctgccttccagcatcgaaaagaccatctccaaggccaagggccagcctagggaaccccaggtttacaccctgcctccaagccaagaggaaatgaccaagaaccaggtgtccctgacctgcctggtcaagggcttctacccttccgatatcgccgtggaatgggagagcaatggccagcctgagaacaactacaagaccacacctcctgtgctggactccgacggctccttctttctgtactcccgcctgaccgtggacaagtccagatggcaagagggcaacgtgttctcctgctctgtgctgcacgaggccctgcacaatcactacacccagaagtccctgtctctgtcccttggcggtggcggaggatctggcggaggcggatctattacatgccctcctccaatgtccgtggaacacgccgacatctgggtcaagtcctacagcctgtactccagagagcggtacatctgcaactccggcttcaagagaaaggccggcacctctagcctgaccgagtgcgtgctgaacaaggccaccaatgtggcccactggacaacccctagcctgaagtgtattagaggcggcggaggaagcggtggcggcggtagcggaggtggtggttctggtggtggcggttctgctcctacctcctccagcaccaagaaaacccagctgcagttggagcatctgctgctggacctgcagatgatcctgaacggctccatgcacatcgacgctaccctgtacaccgagtccgacgtgcacccttcctgtaaagtgaccgccatgaagtgctttctgctcgagctgcaagtgatctccctggaatccaagaacttccacctgaggcctcgggacctgatcgacaacatcaacgtgatcgtgctggaactgaagggctccaacggcaacgtgaccgagtctggctgtaaagagtgcgaggaactggaagagaagaacatcgtcgagtttctgaaccggtggatcaccttctgccagtccatcatctccacactgacc

SEQ ID NO: 139 - DNA, 1359 bp, synthetic construct
  source 1..1359: mol_type = other DNA
ggatccgccgagtctaagtacggccctccttgtcctccatgtcctgctccagaagctgccggagggcccagtgtgtttctgttccctccaaagcctaaggaccagctgatgatctctcggacccctgaagtgacctgcgtggtggtggatgtgtcccaagaggaccctgaggtgcagttcaattggtacgtggacggcgtggaagtgcacaacgccaagaccaagcctagagaggaacagttcaactccacctacagagtggtgtccgtgctgaccgtgctgcaccaggattggctgaacggcaaagagtacaagtgcaaggtgtccaacaagggcctgccttccagcatcgaaaagaccatctccaaggccaagggccagcctagggaaccccaggtttacaccctgcctccaagccaagaggaaatgaccaagaaccaggtgtccctgacctgcctggtcaagggcttctacccttccgatatcgccgtggaatgggagagcaatggccagcctgagaacaactacaagaccacacctcctgtgctggactccgacggctccttctttctgtactcccgcctgaccgtggacaagtccagatggcaagagggcaacgtgttctcctgctctgtgctgcacgaggccctgcacaatcactacacccagaagtccctgtctctgtcccttggcggtggcggaggatctggcggaggcggatctattacatgccctcctccaatgtccgtggaacacgccgacatctgggtcaagtcctacagcctgtactccagagagcggtacatctgcaactccggcttcaagagaaaggccggcacctctagcctgaccgagtgcgtgctgaacaaggccaccaatgtggcccactggacaacccctagcctgaagtgtattagaggcggcggaggaagcggtggcggcggtagcggaggtggtggttctggtggtggcggttctgctcctacctcctccagcaccaagaaaacccagctgcagttggagcatctgctgctggacctgcagatgatcctgaacggctccatgcacatcgacgctaccctgtacaccgagtccgacgtgcacccttcctgtaaagtgaccgccatgaagtgctttctgctcgagctgcaagtgatctccctggaatccaagaacttccacctgaggcctcgggacctgatctccgacatcaacgtgatcgtgctggaactgaagggctccaacggcaacgtgaccgagtctggctgtaaagagtgcgaggaactggaagagaagaacatcgtcgagtttctgaaccggtggatcaccttctgccagtccatcatctccacactgacc

SEQ ID NO: 140 - DNA, 1359 bp, synthetic construct
  source 1..1359: mol_type = other DNA
ggatccgccgagtctaagtacggccctccttgtcctccatgtcctgctccagaagctgccggagggcccagtgtgtttctgttccctccaaagcctaaggaccagctgatgatctctcggacccctgaagtgacctgcgtggtggtggatgtgtcccaagaggaccctgaggtgcagttcaattggtacgtggacggcgtggaagtgcacaacgccaagaccaagcctagagaggaacagttcaactccacctacagagtggtgtccgtgctgaccgtgctgcaccaggattggctgaacggcaaagagtacaagtgcaaggtgtccaacaagggcctgccttccagcatcgaaaagaccatctccaaggccaagggccagcctagggaaccccaggtttacaccctgcctccaagccaagaggaaatgaccaagaaccaggtgtccctgacctgcctggtcaagggcttctacccttccgatatcgccgtggaatgggagagcaatggccagcctgagaacaactacaagaccacacctcctgtgctggactccgacggctccttctttctgtactcccgcctgaccgtggacaagtccagatggcaagagggcaacgtgttctcctgctctgtgctgcacgaggccctgcacaatcactacacccagaagtccctgtctctgtcccttggcggtggcggaggatctggcggaggcggatctattacatgccctcctccaatgtccgtggaacacgccgacatctgggtcaagtcctacagcctgtactccagagagcggtacatctgcaactccggcttcaagagaaaggccggcacctctagcctgaccgagtgcgtgctgaacaaggccaccaatgtggcccactggacaacccctagcctgaagtgtattagaggcggcggaggaagcggtggcggcggtagcggaggtggtggttctggtggtggcggttctgctcctacctcctccagcaccaagaaaacccagctgcagttggagcatctgctgctggacctgcagatgatcctgaacggctccatgcacatcgacgctaccctgtacaccgagtccgacgtgcacccttcctgtaaagtgaccgccatgaagtgctttctgctcgagctgcaagtgatctccctggaatccaagaacttccacctgaggcctcgggacctgatctccaacatcaacctgatcgtgctggaactgaagggctccaacggcaacgtgaccgagtctggctgtaaagagtgcgaggaactggaagagaagaacatcgtcgagtttctgaaccggtggatcaccttctgccagtccatcatctccacactgacc

SEQ ID NO: 141 - DNA, 1359 bp, synthetic construct
  source 1..1359: mol_type = other DNA
ggatccgccgagtctaagtacggccctccttgtcctccatgtcctgctccagaagctgccggagggcccagtgtgtttctgttccctccaaagcctaaggaccagctgatgatctctcggacccctgaagtgacctgcgtggtggtggatgtgtcccaagaggaccctgaggtgcagttcaattggtacgtggacggcgtggaagtgcacaacgccaagaccaagcctagagaggaacagttcaactccacctacagagtggtgtccgtgctgaccgtgctgcaccaggattggctgaacggcaaagagtacaagtgcaaggtgtccaacaagggcctgccttccagcatcgaaaagaccatctccaaggccaagggccagcctagggaaccccaggtttacaccctgcctccaagccaagaggaaatgaccaagaaccaggtgtccctgacctgcctggtcaagggcttctacccttccgatatcgccgtggaatgggagagcaatggccagcctgagaacaactacaagaccacacctcctgtgctggactccgacggctccttctttctgtactcccgcctgaccgtggacaagtccagatggcaagagggcaacgtgttctcctgctctgtgctgcacgaggccctgcacaatcactacacccagaagtccctgtctctgtcccttggcggtggcggaggatctggcggaggcggatctattacatgccctcctccaatgtccgtggaacacgccgacatctgggtcaagtcctacagcctgtactccagagagcggtacatctgcaactccggcttcaagagaaaggccggcacctctagcctgaccgagtgcgtgctgaacaaggccaccaatgtggcccactggacaacccctagcctgaagtgtattagaggcggcggaggaagcggtggcggcggtagcggaggtggtggttctggtggtggcggttctgctcctacctcctccagcaccaagaaaacccagctgcagttggagcatctgctgctggacctgcagatgatcctgaacggctccatgcacatcgacgctaccctgtacaccgagtccgacgtgcacccttcctgtaaagtgaccgccatgaagtgctttctgctcgagctgcaagtgatctccctggaatccaagaacttccacctgaggcctcgggacttcatcgacgacatcaacctgatcgtgctggaactgaagggctccaacggcaacgtgaccgagtctggctgtaaagagtgcgaggaactggaagagaagaacatcgtcgagtttctgaaccggtggatcaccttctgccagtccatcatctccacactgacc

SEQ ID NO: 142 - DNA, 1359 bp, synthetic construct
  source 1..1359: mol_type = other DNA
ggatccgccgagtctaagtacggccctccttgtcctccatgtcctgctccagaagctgccggagggcccagtgtgtttctgttccctccaaagcctaaggaccagctgatgatctctcggacccctgaagtgacctgcgtggtggtggatgtgtcccaagaggaccctgaggtgcagttcaattggtacgtggacggcgtggaagtgcacaacgccaagaccaagcctagagaggaacagttcaactccacctacagagtggtgtccgtgctgaccgtgctgcaccaggattggctgaacggcaaagagtacaagtgcaaggtgtccaacaagggcctgccttccagcatcgaaaagaccatctccaaggccaagggccagcctagggaaccccaggtttacaccctgcctccaagccaagaggaaatgaccaagaaccaggtgtccctgacctgcctggtcaagggcttctacccttccgatatcgccgtggaatgggagagcaatggccagcctgagaacaactacaagaccacacctcctgtgctggactccgacggctccttctttctgtactcccgcctgaccgtggacaagtccagatggcaagagggcaacgtgttctcctgctctgtgctgcacgaggccctgcacaatcactacacccagaagtccctgtctctgtcccttggcggtggcggaggatctggcggaggcggatctattacatgccctcctccaatgtccgtggaacacgccgacatctgggtcaagtcctacagcctgtactccagagagcggtacatctgcaactccggcttcaagagaaaggccggcacctctagcctgaccgagtgcgtgctgaacaaggccaccaatgtggcccactggacaacccctagcctgaagtgtattagaggcggcggaggaagcggtggcggcggtagcggaggtggtggttctggtggtggcggttctgctcctacctcctccagcaccaagaaaacccagctgcagttggagcatctgctgctggacctgcagatgatcctgaacggctccatgcacatcgacgctaccctgtacaccgagtccgacgtgcacccttcctgtaaagtgaccgccatgaagtgctttctgctcgagctgcaagtgatctccctggaatccaagaacttccacctgaggccaagagagctgatcgacgacatcaacctgatcgtgctggaactgaagggctccaacggcaacgtgaccgagtctggctgtaaagagtgcgaggaactggaagagaagaacatcgtcgagtttctgaaccggtggatcaccttctgccagtccatcatctccacactgacc

SEQ ID NO: 143 - DNA, 1359 bp, synthetic construct
  source 1..1359: mol_type = other DNA
ggatccgccgagtctaagtacggccctccttgtcctccatgtcctgctccagaagctgccggagggcccagtgtgtttctgttccctccaaagcctaaggaccagctgatgatctctcggacccctgaagtgacctgcgtggtggtggatgtgtcccaagaggaccctgaggtgcagttcaattggtacgtggacggcgtggaagtgcacaacgccaagaccaagcctagagaggaacagttcaactccacctacagagtggtgtccgtgctgaccgtgctgcaccaggattggctgaacggcaaagagtacaagtgcaaggtgtccaacaagggcctgccttccagcatcgaaaagaccatctccaaggccaagggccagcctagggaaccccaggtttacaccctgcctccaagccaagaggaaatgaccaagaaccaggtgtccctgacctgcctggtcaagggcttctacccttccgatatcgccgtggaatgggagagcaatggccagcctgagaacaactacaagaccacacctcctgtgctggactccgacggctccttctttctgtactcccgcctgaccgtggacaagtccagatggcaagagggcaacgtgttctcctgctctgtgctgcacgaggccctgcacaatcactacacccagaagtccctgtctctgtcccttggcggtggcggaggatctggcggaggcggatctattacatgccctcctccaatgtccgtggaacacgccgacatctgggtcaagtcctacagcctgtactccagagagcggtacatctgcaactccggcttcaagagaaaggccggcacctctagcctgaccgagtgcgtgctgaacaaggccaccaatgtggcccactggacaacccctagcctgaagtgtattagaggcggcggaggaagcggtggcggcggtagcggaggtggtggttctggtggtggcggttctgctcctacctcctccagcaccaagaaaacccagctgcagttggagcatctgctgctggacctgcagatgatcctgaacggctccatgcacatcgacgctaccctgtacaccgagtccgacgtgcacccttcctgtaaagtgaccgccatgaagtgctttctgctcgagctgcaagtgatctccctggaatccaagaacttccacctgaggccaagagagttcatctccgacatcaacctgatcgtgctggaactgaagggctccaacggcaacgtgaccgagtctggctgtaaagagtgcgaggaactggaagagaagaacatcgtcgagtttctgaaccggtggatcaccttctgccagtccatcatctccacactgacc

SEQ ID NO: 144 - DNA, 1359 bp, synthetic construct
  source 1..1359: mol_type = other DNA
ggatccgccgagtctaagtacggccctccttgtcctccatgtcctgctccagaagctgccggagggcccagtgtgtttctgttccctccaaagcctaaggaccagctgatgatctctcggacccctgaagtgacctgcgtggtggtggatgtgtcccaagaggaccctgaggtgcagttcaattggtacgtggacggcgtggaagtgcacaacgccaagaccaagcctagagaggaacagttcaactccacctacagagtggtgtccgtgctgaccgtgctgcaccaggattggctgaacggcaaagagtacaagtgcaaggtgtccaacaagggcctgccttccagcatcgaaaagaccatctccaaggccaagggccagcctagggaaccccaggtttacaccctgcctccaagccaagaggaaatgaccaagaaccaggtgtccctgacctgcctggtcaagggcttctacccttccgatatcgccgtggaatgggagagcaatggccagcctgagaacaactacaagaccacacctcctgtgctggactccgacggctccttctttctgtactcccgcctgaccgtggacaagtccagatggcaagagggcaacgtgttctcctgctctgtgctgcacgaggccctgcacaatcactacacccagaagtccctgtctctgtcccttggcggtggcggaggatctggcggaggcggatctattacatgccctcctccaatgtccgtggaacacgccgacatctgggtcaagtcctacagcctgtactccagagagcggtacatctgcaactccggcttcaagagaaaggccggcacctctagcctgaccgagtgcgtgctgaacaaggccaccaatgtggcccactggacaacccctagcctgaagtgtattagaggcggcggaggaagcggtggcggcggtagcggaggtggtggttctggtggtggcggttctgctcctacctcctccagcaccaagaaaacccagctgcagttggagcatctgctgctggacctgcagatgatcctgaacggctccatgcacatcgacgctaccctgtacaccgagtccgacgtgcacccttcctgtaaagtgaccgccatgaagtgctttctgctcgagctgcaagtgatctccctggaatccaagaacttccacctgaggccaagagagttcatcgacaacatcaacctgatcgtcctggaactgaagggctccaacggcaacgtgaccgagtctggctgtaaagagtgcgaggaactggaagagaagaacatcgtcgagtttctgaaccggtggatcaccttctgccagtccatcatctccacactgacc

SEQ ID NO: 145 - DNA, 1359 bp, synthetic construct
  source 1..1359: mol_type = other DNA
ggatccgccgagtctaagtacggccctccttgtcctccatgtcctgctccagaagctgccggagggcccagtgtgtttctgttccctccaaagcctaaggaccagctgatgatctctcggacccctgaagtgacctgcgtggtggtggatgtgtcccaagaggaccctgaggtgcagttcaattggtacgtggacggcgtggaagtgcacaacgccaagaccaagcctagagaggaacagttcaactccacctacagagtggtgtccgtgctgaccgtgctgcaccaggattggctgaacggcaaagagtacaagtgcaaggtgtccaacaagggcctgccttccagcatcgaaaagaccatctccaaggccaagggccagcctagggaaccccaggtttacaccctgcctccaagccaagaggaaatgaccaagaaccaggtgtccctgacctgcctggtcaagggcttctacccttccgatatcgccgtggaatgggagagcaatggccagcctgagaacaactacaagaccacacctcctgtgctggactccgacggctccttctttctgtactcccgcctgaccgtggacaagtccagatggcaagagggcaacgtgttctcctgctctgtgctgcacgaggccctgcacaatcactacacccagaagtccctgtctctgtcccttggcggtggcggaggatctggcggaggcggatctattacatgccctcctccaatgtccgtggaacacgccgacatctgggtcaagtcctacagcctgtactccagagagcggtacatctgcaactccggcttcaagagaaaggccggcacctctagcctgaccgagtgcgtgctgaacaaggccaccaatgtggcccactggacaacccctagcctgaagtgtattagaggcggcggaggaagcggtggcggcggtagcggaggtggtggttctggtggtggcggttctgctcctacctcctccagcaccaagaaaacccagctgcagttggagcatctgctgctggacctgcagatgatcctgaacggctccatgcacatcgacgctaccctgtacaccgagtccgacgtgcacccttcctgtaaagtgaccgccatgaagtgctttctgctcgagctgcaagtgatctccctggaatccaagaacttccacctgaggccaagagagttcatcgacgacatcaacgtgatcgtgctggaactgaagggctccaacggcaacgtgaccgagtctggctgtaaagagtgcgaggaactggaagagaagaacatcgtcgagtttctgaaccggtggatcaccttctgccagtccatcatctccacactgacc

SEQ ID NO: 146 - DNA, 1359 bp, synthetic construct
  source 1..1359: mol_type = other DNA
ggatccgccgagtctaagtacggccctccttgtcctccatgtcctgctccagaagctgccggagggcccagtgtgtttctgttccctccaaagcctaaggaccagctgatgatctctcggacccctgaagtgacctgcgtggtggtggatgtgtcccaagaggaccctgaggtgcagttcaattggtacgtggacggcgtggaagtgcacaacgccaagaccaagcctagagaggaacagttcaactccacctacagagtggtgtccgtgctgaccgtgctgcaccaggattggctgaacggcaaagagtacaagtgcaaggtgtccaacaagggcctgccttccagcatcgaaaagaccatctccaaggccaagggccagcctagggaaccccaggtttacaccctgcctccaagccaagaggaaatgaccaagaaccaggtgtccctgacctgcctggtcaagggcttctacccttccgatatcgccgtggaatgggagagcaatggccagcctgagaacaactacaagaccacacctcctgtgctggactccgacggctccttctttctgtactcccgcctgaccgtggacaagtccagatggcaagagggcaacgtgttctcctgctctgtgctgcacgaggccctgcacaatcactacacccagaagtccctgtctctgtcccttggcggtggcggaggatctggcggaggcggatctattacatgccctcctccaatgtccgtggaacacgccgacatctgggtcaagtcctacagcctgtactccagagagcggtacatctgcaactccggcttcaagagaaaggccggcacctctagcctgaccgagtgcgtgctgaacaaggccaccaatgtggcccactggacaacccctagcctgaagtgtattagaggcggcggaggaagcggtggcggcggtagcggaggtggtggttctggtggtggcggttctgctcctacctcctccagcaccaagaaaacccagctgcagttggagcatctgctgctggacctgcagatgatcctgaacggctccatgcacatcgacgctaccctgtacaccgagtccgacgtgcacccttcctgtaaagtgaccgccatgaagtgctttctgctcgagctgcaagtgatctccctggaatccaagaacttccacctgaggccaagagagttcatcgacgacatcaacctgatcgtgctggaactgaagggctccaacggcaacgtgaccgagtctggctgtaaagagtgcgaggaactggaagagaagaacatcgtcgagtttctgaaccggtggatcaccttctgccagtccatcatctccacactgacc

SEQ ID NO: 147 - DNA, 1359 bp, synthetic construct
  source 1..1359: mol_type = other DNA
ggatccgccgagtctaagtacggccctccttgtcctccatgtcctgctccagaagctgccggagggcccagtgtgtttctgttccctccaaagcctaaggaccagctgatgatctctcggacccctgaagtgacctgcgtggtggtggatgtgtcccaagaggaccctgaggtgcagttcaattggtacgtggacggcgtggaagtgcacaacgccaagaccaagcctagagaggaacagttcaactccacctacagagtggtgtccgtgctgaccgtgctgcaccaggattggctgaacggcaaagagtacaagtgcaaggtgtccaacaagggcctgccttccagcatcgaaaagaccatctccaaggccaagggccagcctagggaaccccaggtttacaccctgcctccaagccaagaggaaatgaccaagaaccaggtgtccctgacctgcctggtcaagggcttctacccttccgatatcgccgtggaatgggagagcaatggccagcctgagaacaactacaagaccacacctcctgtgctggactccgacggctccttctttctgtactcccgcctgaccgtggacaagtccagatggcaagagggcaacgtgttctcctgctctgtgctgcacgaggccctgcacaatcactacacccagaagtccctgtctctgtcccttggcggtggcggaggatctggcggaggcggatctattacatgccctcctccaatgtccgtggaacacgccgacatctgggtcaagtcctacagcctgtactccagagagcggtacatctgcaactccggcttcaagagaaaggccggcacctctagcctgaccgagtgcgtgctgaacaaggccaccaatgtggcccactggacaacccctagcctgaagtgtattagaggcggcggaggaagcggtggcggcggtagcggaggtggtggttctggtggtggcggttctgctcctacctcctccagcaccaagaaaacccagctgcagttggagcatctgctgctggacctgcagatgatcctgaacggctccatgcacatcgacgctaccctgtacaccgagtccgacgtgcacccttcctgtaaagtgaccgccatgaagtgctttctgttggagctgcaagtgatctccctggaatccaagaacttccacctgaggcctcgggacctgatcgaaaacatcaacgtgatcgtgctggaactgaagggctccaacggcaacgtgaccgagtctggctgtaaagagtgcgaggaactggaagagaagaacatcgtcgagtttctgaaccggtggatcaccttctgccagtccatcatctccacactgacc

SEQ ID NO: 148 - DNA, 1359 bp, synthetic construct
  source 1..1359: mol_type = other DNA
ggatccgccgagtctaagtacggccctccttgtcctccatgtcctgctccagaagctgccggagggcccagtgtgtttctgttccctccaaagcctaaggaccagctgatgatctctcggacccctgaagtgacctgcgtggtggtggatgtgtcccaagaggaccctgaggtgcagttcaattggtacgtggacggcgtggaagtgcacaacgccaagaccaagcctagagaggaacagttcaactccacctacagagtggtgtccgtgctgaccgtgctgcaccaggattggctgaacggcaaagagtacaagtgcaaggtgtccaacaagggcctgccttccagcatcgaaaagaccatctccaaggccaagggccagcctagggaaccccaggtttacaccctgcctccaagccaagaggaaatgaccaagaaccaggtgtccctgacctgcctggtcaagggcttctacccttccgatatcgccgtggaatgggagagcaatggccagcctgagaacaactacaagaccacacctcctgtgctggactccgacggctccttctttctgtactcccgcctgaccgtggacaagtccagatggcaagagggcaacgtgttctcctgctctgtgctgcacgaggccctgcacaatcactacacccagaagtccctgtctctgtcccttggcggtggcggaggatctggcggaggcggatctattacatgccctcctccaatgtccgtggaacacgccgacatctgggtcaagtcctacagcctgtactccagagagcggtacatctgcaactccggcttcaagagaaaggccggcacctctagcctgaccgagtgcgtgctgaacaaggccaccaatgtggcccactggacaacccctagcctgaagtgtattagaggcggcggaggaagcggtggcggcggtagcggaggtggtggttctggtggtggcggttctgctcctacctcctccagcaccaagaaaacccagctgcagttggagcatctgctgctggacctgcagatgatcctgaacggctccatgcacatcgacgctaccctgtacaccgagtccgacgtgcacccttcctgtaaagtgaccgccatgaagtgctttctgttggagctgcaagtgatctccctggaatccaagaacttccacctgaggcctcgggacctgatcaacaacatcaacgtgatcgtgctggaactgaagggctccaacggcaacgtgaccgagtctggctgtaaagagtgcgaggaactggaagagaagaacatcgtcgagtttctgaaccggtggatcaccttctgccagtccatcatctccacactgacc

SEQ ID NO: 149 - DNA, 1359 bp, synthetic construct
  source 1..1359: mol_type = other DNA
ggatccgccgagtctaagtacggccctccttgtcctccatgtcctgctccagaagctgccggagggcccagtgtgtttctgttccctccaaagcctaaggaccagctgatgatctctcggacccctgaagtgacctgcgtggtggtggatgtgtcccaagaggaccctgaggtgcagttcaattggtacgtggacggcgtggaagtgcacaacgccaagaccaagcctagagaggaacagttcaactccacctacagagtggtgtccgtgctgaccgtgctgcaccaggattggctgaacggcaaagagtacaagtgcaaggtgtccaacaagggcctgccttccagcatcgaaaagaccatctccaaggccaagggccagcctagggaaccccaggtttacaccctgcctccaagccaagaggaaatgaccaagaaccaggtgtccctgacctgcctggtcaagggcttctacccttccgatatcgccgtggaatgggagagcaatggccagcctgagaacaactacaagaccacacctcctgtgctggactccgacggctccttctttctgtactcccgcctgaccgtggacaagtccagatggcaagagggcaacgtgttctcctgctctgtgctgcacgaggccctgcacaatcactacacccagaagtccctgtctctgtcccttggcggtggcggaggatctggcggaggcggatctattacatgccctcctccaatgtccgtggaacacgccgacatctgggtcaagtcctacagcctgtactccagagagcggtacatctgcaactccggcttcaagagaaaggccggcacctctagcctgaccgagtgcgtgctgaacaaggccaccaatgtggcccactggacaacccctagcctgaagtgtattagaggcggcggaggaagcggtggcggcggtagcggaggtggtggttctggtggtggcggttctgctcctacctcctccagcaccaagaaaacccagctgcagttggagcatctgctgctggacctgcagatgatcctgaacggctccatgcacatcgacgctaccctgtacaccgagtccgacgtgcacccttcctgtaaagtgaccgccatgaagtgctttctgttggagctgcaagtgatctccctggaatccaagaacttccacctgaggcctcgggacctgatcaagaacatcaacgtgatcgtgctggaactgaagggctccaacggcaacgtgaccgagtctggctgtaaagagtgcgaggaactggaagagaagaacatcgtcgagtttctgaaccggtggatcaccttctgccagtccatcatctccacactgacc

SEQ ID NO: 150 - DNA, 1359 bp, synthetic construct
  source 1..1359: mol_type = other DNA
ggatccgccgagtctaagtacggccctccttgtcctccatgtcctgctccagaagctgccggagggcccagtgtgtttctgttccctccaaagcctaaggaccagctgatgatctctcggacccctgaagtgacctgcgtggtggtggatgtgtcccaagaggaccctgaggtgcagttcaattggtacgtggacggcgtggaagtgcacaacgccaagaccaagcctagagaggaacagttcaactccacctacagagtggtgtccgtgctgaccgtgctgcaccaggattggctgaacggcaaagagtacaagtgcaaggtgtccaacaagggcctgccttccagcatcgaaaagaccatctccaaggccaagggccagcctagggaaccccaggtttacaccctgcctccaagccaagaggaaatgaccaagaaccaggtgtccctgacctgcctggtcaagggcttctacccttccgatatcgccgtggaatgggagagcaatggccagcctgagaacaactacaagaccacacctcctgtgctggactccgacggctccttctttctgtactcccgcctgaccgtggacaagtccagatggcaagagggcaacgtgttctcctgctctgtgctgcacgaggccctgcacaatcactacacccagaagtccctgtctctgtcccttggcggtggcggaggatctggcggaggcggatctattacatgccctcctccaatgtccgtggaacacgccgacatctgggtcaagtcctacagcctgtactccagagagcggtacatctgcaactccggcttcaagagaaaggccggcacctctagcctgaccgagtgcgtgctgaacaaggccaccaatgtggcccactggacaacccctagcctgaagtgtattagaggcggcggaggaagcggtggcggcggtagcggaggtggtggttctggtggtggcggttctgctcctacctcctccagcaccaagaaaacccagctgcagttggagcatctgctgctggacctgcagatgatcctgaacggctccatgcacatcgacgctaccctgtacaccgagtccgacgtgcacccttcctgtaaagtgaccgccatgaagtgctttctgttggagctgcaagtgatctccctggaatccaagaacttccacctgaggcctcgggacctgatcctcaacatcaacgtgatcgtgctggaactgaagggctccaacggcaacgtgaccgagtctggctgtaaagagtgcgaggaactggaagagaagaacatcgtcgagtttctgaaccggtggatcaccttctgccagtccatcatctccacactgacc

SEQ ID NO: 151 - DNA, 1359 bp, synthetic construct
  source 1..1359: mol_type = other DNA
ggatccgccgagtctaagtacggccctccttgtcctccatgtcctgctccagaagctgccggagggcccagtgtgtttctgttccctccaaagcctaaggaccagctgatgatctctcggacccctgaagtgacctgcgtggtggtggatgtgtcccaagaggaccctgaggtgcagttcaattggtacgtggacggcgtggaagtgcacaacgccaagaccaagcctagagaggaacagttcaactccacctacagagtggtgtccgtgctgaccgtgctgcaccaggattggctgaacggcaaagagtacaagtgcaaggtgtccaacaagggcctgccttccagcatcgaaaagaccatctccaaggccaagggccagcctagggaaccccaggtttacaccctgcctccaagccaagaggaaatgaccaagaaccaggtgtccctgacctgcctggtcaagggcttctacccttccgatatcgccgtggaatgggagagcaatggccagcctgagaacaactacaagaccacacctcctgtgctggactccgacggctccttctttctgtactcccgcctgaccgtggacaagtccagatggcaagagggcaacgtgttctcctgctctgtgctgcacgaggccctgcacaatcactacacccagaagtccctgtctctgtcccttggcggtggcggaggatctggcggaggcggatctattacatgccctcctccaatgtccgtggaacacgccgacatctgggtcaagtcctacagcctgtactccagagagcggtacatctgcaactccggcttcaagagaaaggccggcacctctagcctgaccgagtgcgtgctgaacaaggccaccaatgtggcccactggacaacccctagcctgaagtgtattagaggcggcggaggaagcggtggcggcggtagcggaggtggtggttctggtggtggcggttctgctcctacctcctccagcaccaagaaaacccagctgcagttggagcatctgctgctggacctgcagatgatcctgaacggctccatgcacatcgacgctaccctgtacaccgagtccgacgtgcacccttcctgtaaagtgaccgccatgaagtgctttctgctcgagctgcaagtgatctccctggaatccaagaacttccacctgaggcctcgggacttcatcgacaacatcaacgtgatcgtgctggaactgaagggctccaacggcaacgtgaccgagtctggctgtaaagagtgcgaggaactggaagagaagaacatcgtcgagtttctgaaccggtggatcaccttctgccagtccatcatctccacactgacc

SEQ ID NO: 152 - DNA, 1359 bp, synthetic construct
  source 1..1359: mol_type = other DNA
ggatccgccgagtctaagtacggccctccttgtcctccatgtcctgctccagaagctgccggagggcccagtgtgtttctgttccctccaaagcctaaggaccagctgatgatctctcggacccctgaagtgacctgcgtggtggtggatgtgtcccaagaggaccctgaggtgcagttcaattggtacgtggacggcgtggaagtgcacaacgccaagaccaagcctagagaggaacagttcaactccacctacagagtggtgtccgtgctgaccgtgctgcaccaggattggctgaacggcaaagagtacaagtgcaaggtgtccaacaagggcctgccttccagcatcgaaaagaccatctccaaggccaagggccagcctagggaaccccaggtttacaccctgcctccaagccaagaggaaatgaccaagaaccaggtgtccctgacctgcctggtcaagggcttctacccttccgatatcgccgtggaatgggagagcaatggccagcctgagaacaactacaagaccacacctcctgtgctggactccgacggctccttctttctgtactcccgcctgaccgtggacaagtccagatggcaagagggcaacgtgttctcctgctctgtgctgcacgaggccctgcacaatcactacacccagaagtccctgtctctgtcccttggcggtggcggaggatctggcggaggcggatctattacatgccctcctccaatgtccgtggaacacgccgacatctgggtcaagtcctacagcctgtactccagagagcggtacatctgcaactccggcttcaagagaaaggccggcacctctagcctgaccgagtgcgtgctgaacaaggccaccaatgtggcccactggacaacccctagcctgaagtgtattagaggcggcggaggaagcggtggcggcggtagcggaggtggtggttctggtggtggcggttctgctcctacctcctccagcaccaagaaaacccagctgcagttggagcatctgctgctggacctgcagatgatcctgaacggctccatgcacatcgacgctaccctgtacaccgagtccgacgtgcacccttcctgtaaagtgaccgccatgaagtgctttctgctcgagctgcaagtgatctccctggaatccaagaacttccacctgaggcctcgggacctgatcgacgacatcaacgtgatcgtgctggaactgaagggctccaacggcaacgtgaccgagtctggctgtaaagagtgcgaggaactggaagagaagaacatcgtcgagtttctgaaccggtggatcaccttctgccagtccatcatctccacactgacc

SEQ ID NO: 153 - DNA, 1359 bp, synthetic construct
  source 1..1359: mol_type = other DNA
ggatccgccgagtctaagtacggccctccttgtcctccatgtcctgctccagaagctgccggagggcccagtgtgtttctgttccctccaaagcctaaggaccagctgatgatctctcggacccctgaagtgacctgcgtggtggtggatgtgtcccaagaggaccctgaggtgcagttcaattggtacgtggacggcgtggaagtgcacaacgccaagaccaagcctagagaggaacagttcaactccacctacagagtggtgtccgtgctgaccgtgctgcaccaggattggctgaacggcaaagagtacaagtgcaaggtgtccaacaagggcctgccttccagcatcgaaaagaccatctccaaggccaagggccagcctagggaaccccaggtttacaccctgcctccaagccaagaggaaatgaccaagaaccaggtgtccctgacctgcctggtcaagggcttctacccttccgatatcgccgtggaatgggagagcaatggccagcctgagaacaactacaagaccacacctcctgtgctggactccgacggctccttctttctgtactcccgcctgaccgtggacaagtccagatggcaagagggcaacgtgttctcctgctctgtgctgcacgaggccctgcacaatcactacacccagaagtccctgtctctgtcccttggcggtggcggaggatctggcggaggcggatctattacatgccctcctccaatgtccgtggaacacgccgacatctgggtcaagtcctacagcctgtactccagagagcggtacatctgcaactccggcttcaagagaaaggccggcacctctagcctgaccgagtgcgtgctgaacaaggccaccaatgtggcccactggacaacccctagcctgaagtgtattagaggcggcggaggaagcggtggcggcggtagcggaggtggtggttctggtggtggcggttctgctcctacctcctccagcaccaagaaaacccagctgcagttggagcatctgctgctggacctgcagatgatcctgaacggctccatgcacatcgacgctaccctgtacaccgagtccgacgtgcacccttcctgtaaagtgaccgccatgaagtgctttctgctcgagctgcaagtgatctccctggaatccaagaacttccacctgaggcctcgggacctgatcgacaacatcaacctgatcgtgctggaactgaagggctccaacggcaacgtgaccgagtctggctgtaaagagtgcgaggaactggaagagaagaacatcgtcgagtttctgaaccggtggatcaccttctgccagtccatcatctccacactgacc

SEQ ID NO: 154 - DNA, 1359 bp, synthetic construct
  source 1..1359: mol_type = other DNA
ggatccgccgagtctaagtacggccctccttgtcctccatgtcctgctccagaagctgccggagggcccagtgtgtttctgttccctccaaagcctaaggaccagctgatgatctctcggacccctgaagtgacctgcgtggtggtggatgtgtcccaagaggaccctgaggtgcagttcaattggtacgtggacggcgtggaagtgcacaacgccaagaccaagcctagagaggaacagttcaactccacctacagagtggtgtccgtgctgaccgtgctgcaccaggattggctgaacggcaaagagtacaagtgcaaggtgtccaacaagggcctgccttccagcatcgaaaagaccatctccaaggccaagggccagcctagggaaccccaggtttacaccctgcctccaagccaagaggaaatgaccaagaaccaggtgtccctgacctgcctggtcaagggcttctacccttccgatatcgccgtggaatgggagagcaatggccagcctgagaacaactacaagaccacacctcctgtgctggactccgacggctccttctttctgtactcccgcctgaccgtggacaagtccagatggcaagagggcaacgtgttctcctgctctgtgctgcacgaggccctgcacaatcactacacccagaagtccctgtctctgtcccttggcggtggcggaggatctggcggaggcggatctattacatgccctcctccaatgtccgtggaacacgccgacatctgggtcaagtcctacagcctgtactccagagagcggtacatctgcaactccggcttcaagagaaaggccggcacctctagcctgaccgagtgcgtgctgaacaaggccaccaatgtggcccactggacaacccctagcctgaagtgtattagaggcggcggaggaagcggtggcggcggtagcggaggtggtggttctggtggtggcggttctgctcctacctcctccagcaccaagaaaacccagctgcagttggagcatctgctgctggacctgcagatgatcctgaacggctccatgcacatcgacgctaccctgtacaccgagtccgacgtgcacccttcctgtaaagtgaccgccatgaagtgctttctgctcgagctgcaagtgatctccctggaatccaagaacttccacctgaggcctcgggacttcatcgacgacatcaacgtgatcgtgctggaactgaagggctccaacggcaacgtgaccgagtctggctgtaaagagtgcgaggaactggaagagaagaacatcgtcgagtttctgaaccggtggatcaccttctgccagtccatcatctccacactgacc

SEQ ID NO: 155 - DNA, 1359 bp, synthetic construct
  source 1..1359: mol_type = other DNA
ggatccgccgagtctaagtacggccctccttgtcctccatgtcctgctccagaagctgccggagggcccagtgtgtttctgttccctccaaagcctaaggaccagctgatgatctctcggacccctgaagtgacctgcgtggtggtggatgtgtcccaagaggaccctgaggtgcagttcaattggtacgtggacggcgtggaagtgcacaacgccaagaccaagcctagagaggaacagttcaactccacctacagagtggtgtccgtgctgaccgtgctgcaccaggattggctgaacggcaaagagtacaagtgcaaggtgtccaacaagggcctgccttccagcatcgaaaagaccatctccaaggccaagggccagcctagggaaccccaggtttacaccctgcctccaagccaagaggaaatgaccaagaaccaggtgtccctgacctgcctggtcaagggcttctacccttccgatatcgccgtggaatgggagagcaatggccagcctgagaacaactacaagaccacacctcctgtgctggactccgacggctccttctttctgtactcccgcctgaccgtggacaagtccagatggcaagagggcaacgtgttctcctgctctgtgctgcacgaggccctgcacaatcactacacccagaagtccctgtctctgtcccttggcggtggcggaggatctggcggaggcggatctattacatgccctcctccaatgtccgtggaacacgccgacatctgggtcaagtcctacagcctgtactccagagagcggtacatctgcaactccggcttcaagagaaaggccggcacctctagcctgaccgagtgcgtgctgaacaaggccaccaatgtggcccactggacaacccctagcctgaagtgtattagaggcggcggaggaagcggtggcggcggtagcggaggtggtggttctggtggtggcggttctgctcctacctcctccagcaccaagaaaacccagctgcagttggagcatctgctgctggacctgcagatgatcctgaacggctccatgcacatcgacgctaccctgtacaccgagtccgacgtgcacccttcctgtaaagtgaccgccatgaagtgctttctgctcgagctgcaagtgatctccctggaatccaagaacttccacctgaggcctcgggacctgatcgacgacatcaacctgatcgtgctggaactgaagggctccaacggcaacgtgaccgagtctggctgtaaagagtgcgaggaactggaagagaagaacatcgtcgagtttctgaaccggtggatcaccttctgccagtccatcatctccacactgacc

SEQ ID NO: 156 - DNA, 1359 bp, synthetic construct
  source 1..1359: mol_type = other DNA
ggatccgccgagtctaagtacggccctccttgtcctccatgtcctgctccagaagctgccggagggcccagtgtgtttctgttccctccaaagcctaaggaccagctgatgatctctcggacccctgaagtgacctgcgtggtggtggatgtgtcccaagaggaccctgaggtgcagttcaattggtacgtggacggcgtggaagtgcacaacgccaagaccaagcctagagaggaacagttcaactccacctacagagtggtgtccgtgctgaccgtgctgcaccaggattggctgaacggcaaagagtacaagtgcaaggtgtccaacaagggcctgccttccagcatcgaaaagaccatctccaaggccaagggccagcctagggaaccccaggtttacaccctgcctccaagccaagaggaaatgaccaagaaccaggtgtccctgacctgcctggtcaagggcttctacccttccgatatcgccgtggaatgggagagcaatggccagcctgagaacaactacaagaccacacctcctgtgctggactccgacggctccttctttctgtactcccgcctgaccgtggacaagtccagatggcaagagggcaacgtgttctcctgctctgtgctgcacgaggccctgcacaatcactacacccagaagtccctgtctctgtcccttggcggtggcggaggatctggcggaggcggatctattacatgccctcctccaatgtccgtggaacacgccgacatctgggtcaagtcctacagcctgtactccagagagcggtacatctgcaactccggcttcaagagaaaggccggcacctctagcctgaccgagtgcgtgctgaacaaggccaccaatgtggcccactggacaacccctagcctgaagtgtattagaggcggcggaggaagcggtggcggcggtagcggaggtggtggttctggtggtggcggttctgctcctacctcctccagcaccaagaaaacccagctgcagttggagcatctgctgctggacctgcagatgatcctgaacggctccatgcacatcgacgctaccctgtacaccgagtccgacgtgcacccttcctgtaaagtgaccgccatgaagtgctttctgctcgagctgcaagtgatctccctggaatccaagaacttccacctgaggcctcgggacttcatcgacaacatcaacctgatcgtgctggaactgaagggctccaacggcaacgtgaccgagtctggctgtaaagagtgcgaggaactggaagagaagaacatcgtcgagtttctgaaccggtggatcaccttctgccagtccatcatctccacactgacc

SEQ ID NO: 157 - DNA, 1359 bp, synthetic construct
  source 1..1359: mol_type = other DNA
gctcctacctcctccagcaccaagaaaacccagctgcagttggagcatctgctgctggacctgcagatgatcctgaacggctccatgcacatcgacgctaccctgtacaccgagtccgacgtgcacccttcctgtaaagtgaccgccatgaagtgctttctgttggagctgcaagtgatctccctggaatccaagaacttccacctgaggcctcgggacctgatctccaacatcaacgtgatcgtgctggaactgaagggctccaacggcaacgtgaccgagtctggctgtaaagagtgcgaggaactggaagagaagaacatcgtcgagtttctgaaccggtggatcaccttctgccagtccatcatctccacactgaccggcggcggaggaagcggtggcggcggtagcggaggtggtggttctggtggtggcggttctattacatgccctcctccaatgtccgtggaacacgccgacatctgggtcaagtcctacagcctgtactccagagagcggtacatctgcaactccggcttcaagagaaaggccggcacctctagcctgaccgagtgcgtgctgaacaaggccaccaatgtggcccactggacaacccctagcctgaagtgtattagaggtggcggaggatctggcggaggcggatctggatccgccgagtctaagtacggccctccttgtcctccatgtcctgctccagaagctgccggagggcccagtgtgtttctgttccctccaaagcctaaggaccagctgatgatctctcggacccctgaagtgacctgcgtggtggtggatgtgtcccaagaggaccctgaggtgcagttcaattggtacgtggacggcgtggaagtgcacaacgccaagaccaagcctagagaggaacagttcaactccacctacagagtggtgtccgtgctgaccgtgctgcaccaggattggctgaacggcaaagagtacaagtgcaaggtgtccaacaagggcctgccttccagcatcgaaaagaccatctccaaggccaagggccagcctagggaaccccaggtttacaccctgcctccaagccaagaggaaatgaccaagaaccaggtgtccctgacctgcctggtcaagggcttctacccttccgatatcgccgtggaatgggagagcaatggccagcctgagaacaactacaagaccacacctcctgtgctggactccgacggctccttctttctgtactcccgcctgaccgtggacaagtccagatggcaagagggcaacgtgttctcctgctctgtgctgcacgaggccctgcacaatcactacacccagaagtccctgtctctgtcccttggc

SEQ ID NO: 158 - DNA, 1359 bp, synthetic construct
  source 1..1359: mol_type = other DNA
gctcctacctcctccagcaccaagaaaacccagctgcagttggagcatctgctgctggacctgcagatgatcctgaacggctccatgcacatcgacgctaccctgtacaccgagtccgacgtgcacccttcctgtaaagtgaccgccatgaagtgctttctgctcgagctgcaagtgatctccctggaatccaagaacttccacctgaggccaagagagctgatctccaacatcaacgtgatcgtgctggaactgaagggctccaacggcaacgtgaccgagtctggctgtaaagagtgcgaggaactggaagagaagaacatcgtcgagtttctgaaccggtggatcaccttctgccagtccatcatctccacactgaccggcggcggaggaagcggtggcggcggtagcggaggtggtggttctggtggtggcggttctattacatgccctcctccaatgtccgtggaacacgccgacatctgggtcaagtcctacagcctgtactccagagagcggtacatctgcaactccggcttcaagagaaaggccggcacctctagcctgaccgagtgcgtgctgaacaaggccaccaatgtggcccactggacaacccctagcctgaagtgtattagaggtggcggaggatctggcggaggcggatctggatccgccgagtctaagtacggccctccttgtcctccatgtcctgctccagaagctgccggagggcccagtgtgtttctgttccctccaaagcctaaggaccagctgatgatctctcggacccctgaagtgacctgcgtggtggtggatgtgtcccaagaggaccctgaggtgcagttcaattggtacgtggacggcgtggaagtgcacaacgccaagaccaagcctagagaggaacagttcaactccacctacagagtggtgtccgtgctgaccgtgctgcaccaggattggctgaacggcaaagagtacaagtgcaaggtgtccaacaagggcctgccttccagcatcgaaaagaccatctccaaggccaagggccagcctagggaaccccaggtttacaccctgcctccaagccaagaggaaatgaccaagaaccaggtgtccctgacctgcctggtcaagggcttctacccttccgatatcgccgtggaatgggagagcaatggccagcctgagaacaactacaagaccacacctcctgtgctggactccgacggctccttctttctgtactcccgcctgaccgtggacaagtccagatggcaagagggcaacgtgttctcctgctctgtgctgcacgaggccctgcacaatcactacacccagaagtccctgtctctgtcccttggc

SEQ ID NO: 159 - DNA, 1359 bp, synthetic construct
  source 1..1359: mol_type = other DNA
gctcctacctcctccagcaccaagaaaacccagctgcagttggagcatctgctgctggacctgcagatgatcctgaacggctccatgcacatcgacgctaccctgtacaccgagtccgacgtgcacccttcctgtaaagtgaccgccatgaagtgctttctgctcgagctgcaagtgatctccctggaatccaagaacttccacctgaggcctcgggacttcatctccaacatcaacgtgatcgtgctggaactgaagggctccaacggcaacgtgaccgagtctggctgtaaagagtgcgaggaactggaagagaagaacatcgtcgagtttctgaaccggtggatcaccttctgccagtccatcatctccacactgaccggcggcggaggaagcggtggcggcggtagcggaggtggtggttctggtggtggcggttctattacatgccctcctccaatgtccgtggaacacgccgacatctgggtcaagtcctacagcctgtactccagagagcggtacatctgcaactccggcttcaagagaaaggccggcacctctagcctgaccgagtgcgtgctgaacaaggccaccaatgtggcccactggacaacccctagcctgaagtgtattagaggtggcggaggatctggcggaggcggatctggatccgccgagtctaagtacggccctccttgtcctccatgtcctgctccagaagctgccggagggcccagtgtgtttctgttccctccaaagcctaaggaccagctgatgatctctcggacccctgaagtgacctgcgtggtggtggatgtgtcccaagaggaccctgaggtgcagttcaattggtacgtggacggcgtggaagtgcacaacgccaagaccaagcctagagaggaacagttcaactccacctacagagtggtgtccgtgctgaccgtgctgcaccaggattggctgaacggcaaagagtacaagtgcaaggtgtccaacaagggcctgccttccagcatcgaaaagaccatctccaaggccaagggccagcctagggaaccccaggtttacaccctgcctccaagccaagaggaaatgaccaagaaccaggtgtccctgacctgcctggtcaagggcttctacccttccgatatcgccgtggaatgggagagcaatggccagcctgagaacaactacaagaccacacctcctgtgctggactccgacggctccttctttctgtactcccgcctgaccgtggacaagtccagatggcaagagggcaacgtgttctcctgctctgtgctgcacgaggccctgcacaatcactacacccagaagtccctgtctctgtcccttggc

SEQ ID NO: 160 - DNA, 1359 bp, synthetic construct
  source 1..1359: mol_type = other DNA
gctcctacctcctccagcaccaagaaaacccagctgcagttggagcatctgctgctggacctgcagatgatcctgaacggctccatgcacatcgacgctaccctgtacaccgagtccgacgtgcacccttcctgtaaagtgaccgccatgaagtgctttctgctcgagctgcaagtgatctccctggaatccaagaacttccacctgaggcctcgggacctgatcgacaacatcaacgtgatcgtgctggaactgaagggctccaacggcaacgtgaccgagtctggctgtaaagagtgcgaggaactggaagagaagaacatcgtcgagtttctgaaccggtggatcaccttctgccagtccatcatctccacactgaccggcggcggaggaagcggtggcggcggtagcggaggtggtggttctggtggtggcggttctattacatgccctcctccaatgtccgtggaacacgccgacatctgggtcaagtcctacagcctgtactccagagagcggtacatctgcaactccggcttcaagagaaaggccggcacctctagcctgaccgagtgcgtgctgaacaaggccaccaatgtggcccactggacaacccctagcctgaagtgtattagaggtggcggaggatctggcggaggcggatctggatccgccgagtctaagtacggccctccttgtcctccatgtcctgctccagaagctgccggagggcccagtgtgtttctgttccctccaaagcctaaggaccagctgatgatctctcggacccctgaagtgacctgcgtggtggtggatgtgtcccaagaggaccctgaggtgcagttcaattggtacgtggacggcgtggaagtgcacaacgccaagaccaagcctagagaggaacagttcaactccacctacagagtggtgtccgtgctgaccgtgctgcaccaggattggctgaacggcaaagagtacaagtgcaaggtgtccaacaagggcctgccttccagcatcgaaaagaccatctccaaggccaagggccagcctagggaaccccaggtttacaccctgcctccaagccaagaggaaatgaccaagaaccaggtgtccctgacctgcctggtcaagggcttctacccttccgatatcgccgtggaatgggagagcaatggccagcctgagaacaactacaagaccacacctcctgtgctggactccgacggctccttctttctgtactcccgcctgaccgtggacaagtccagatggcaagagggcaacgtgttctcctgctctgtgctgcacgaggccctgcacaatcactacacccagaagtccctgtctctgtcccttggc

SEQ ID NO: 161 - DNA, 1359 bp, synthetic construct
  source 1..1359: mol_type = other DNA
gctcctacctcctccagcaccaagaaaacccagctgcagttggagcatctgctgctggacctgcagatgatcctgaacggctccatgcacatcgacgctaccctgtacaccgagtccgacgtgcacccttcctgtaaagtgaccgccatgaagtgctttctgctcgagctgcaagtgatctccctggaatccaagaacttccacctgaggcctcgggacctgatctccgacatcaacgtgatcgtgctggaactgaagggctccaacggcaacgtgaccgagtctggctgtaaagagtgcgaggaactggaagagaagaacatcgtcgagtttctgaaccggtggatcaccttctgccagtccatcatctccacactgaccggcggcggaggaagcggtggcggcggtagcggaggtggtggttctggtggtggcggttctattacatgccctcctccaatgtccgtggaacacgccgacatctgggtcaagtcctacagcctgtactccagagagcggtacatctgcaactccggcttcaagagaaaggccggcacctctagcctgaccgagtgcgtgctgaacaaggccaccaatgtggcccactggacaacccctagcctgaagtgtattagaggtggcggaggatctggcggaggcggatctggatccgccgagtctaagtacggccctccttgtcctccatgtcctgctccagaagctgccggagggcccagtgtgtttctgttccctccaaagcctaaggaccagctgatgatctctcggacccctgaagtgacctgcgtggtggtggatgtgtcccaagaggaccctgaggtgcagttcaattggtacgtggacggcgtggaagtgcacaacgccaagaccaagcctagagaggaacagttcaactccacctacagagtggtgtccgtgctgaccgtgctgcaccaggattggctgaacggcaaagagtacaagtgcaaggtgtccaacaagggcctgccttccagcatcgaaaagaccatctccaaggccaagggccagcctagggaaccccaggtttacaccctgcctccaagccaagaggaaatgaccaagaaccaggtgtccctgacctgcctggtcaagggcttctacccttccgatatcgccgtggaatgggagagcaatggccagcctgagaacaactacaagaccacacctcctgtgctggactccgacggctccttctttctgtactcccgcctgaccgtggacaagtccagatggcaagagggcaacgtgttctcctgctctgtgctgcacgaggccctgcacaatcactacacccagaagtccctgtctctgtcccttggc

SEQ ID NO: 162 - DNA, 1359 bp, synthetic construct
  source 1..1359: mol_type = other DNA
gctcctacctcctccagcaccaagaaaacccagctgcagttggagcatctgctgctggacctgcagatgatcctgaacggctccatgcacatcgacgctaccctgtacaccgagtccgacgtgcacccttcctgtaaagtgaccgccatgaagtgctttctgctcgagctgcaagtgatctccctggaatccaagaacttccacctgaggcctcgggacctgatctccaacatcaacctgatcgtgctggaactgaagggctccaacggcaacgtgaccgagtctggctgtaaagagtgcgaggaactggaagagaagaacatcgtcgagtttctgaaccggtggatcaccttctgccagtccatcatctccacactgaccggcggcggaggaagcggtggcggcggtagcggaggtggtggttctggtggtggcggttctattacatgccctcctccaatgtccgtggaacacgccgacatctgggtcaagtcctacagcctgtactccagagagcggtacatctgcaactccggcttcaagagaaaggccggcacctctagcctgaccgagtgcgtgctgaacaaggccaccaatgtggcccactggacaacccctagcctgaagtgtattagaggtggcggaggatctggcggaggcggatctggatccgccgagtctaagtacggccctccttgtcctccatgtcctgctccagaagctgccggagggcccagtgtgtttctgttccctccaaagcctaaggaccagctgatgatctctcggacccctgaagtgacctgcgtggtggtggatgtgtcccaagaggaccctgaggtgcagttcaattggtacgtggacggcgtggaagtgcacaacgccaagaccaagcctagagaggaacagttcaactccacctacagagtggtgtccgtgctgaccgtgctgcaccaggattggctgaacggcaaagagtacaagtgcaaggtgtccaacaagggcctgccttccagcatcgaaaagaccatctccaaggccaagggccagcctagggaaccccaggtttacaccctgcctccaagccaagaggaaatgaccaagaaccaggtgtccctgacctgcctggtcaagggcttctacccttccgatatcgccgtggaatgggagagcaatggccagcctgagaacaactacaagaccacacctcctgtgctggactccgacggctccttctttctgtactcccgcctgaccgtggacaagtccagatggcaagagggcaacgtgttctcctgctctgtgctgcacgaggccctgcacaatcactacacccagaagtccctgtctctgtcccttggc

SEQ ID NO: 163 - DNA, 1359 bp, synthetic construct
  source 1..1359: mol_type = other DNA
gctcctacctcctccagcaccaagaaaacccagctgcagttggagcatctgctgctggacctgcagatgatcctgaacggctccatgcacatcgacgctaccctgtacaccgagtccgacgtgcacccttcctgtaaagtgaccgccatgaagtgctttctgctcgagctgcaagtgatctccctggaatccaagaacttccacctgaggcctcgggacttcatcgacgacatcaacctgatcgtgctggaactgaagggctccaacggcaacgtgaccgagtctggctgtaaagagtgcgaggaactggaagagaagaacatcgtcgagtttctgaaccggtggatcaccttctgccagtccatcatctccacactgaccggcggcggaggaagcggtggcggcggtagcggaggtggtggttctggtggtggcggttctattacatgccctcctccaatgtccgtggaacacgccgacatctgggtcaagtcctacagcctgtactccagagagcggtacatctgcaactccggcttcaagagaaaggccggcacctctagcctgaccgagtgcgtgctgaacaaggccaccaatgtggcccactggacaacccctagcctgaagtgtattagaggtggcggaggatctggcggaggcggatctggatccgccgagtctaagtacggccctccttgtcctccatgtcctgctccagaagctgccggagggcccagtgtgtttctgttccctccaaagcctaaggaccagctgatgatctctcggacccctgaagtgacctgcgtggtggtggatgtgtcccaagaggaccctgaggtgcagttcaattggtacgtggacggcgtggaagtgcacaacgccaagaccaagcctagagaggaacagttcaactccacctacagagtggtgtccgtgctgaccgtgctgcaccaggattggctgaacggcaaagagtacaagtgcaaggtgtccaacaagggcctgccttccagcatcgaaaagaccatctccaaggccaagggccagcctagggaaccccaggtttacaccctgcctccaagccaagaggaaatgaccaagaaccaggtgtccctgacctgcctggtcaagggcttctacccttccgatatcgccgtggaatgggagagcaatggccagcctgagaacaactacaagaccacacctcctgtgctggactccgacggctccttctttctgtactcccgcctgaccgtggacaagtccagatggcaagagggcaacgtgttctcctgctctgtgctgcacgaggccctgcacaatcactacacccagaagtccctgtctctgtcccttggc

SEQ ID NO: 164 - DNA, 1359 bp, synthetic construct
  source 1..1359: mol_type = other DNA
gctcctacctcctccagcaccaagaaaacccagctgcagttggagcatctgctgctggacctgcagatgatcctgaacggctccatgcacatcgacgctaccctgtacaccgagtccgacgtgcacccttcctgtaaagtgaccgccatgaagtgctttctgctcgagctgcaagtgatctccctggaatccaagaacttccacctgaggccaagagagctgatcgacgacatcaacctgatcgtgctggaactgaagggctccaacggcaacgtgaccgagtctggctgtaaagagtgcgaggaactggaagagaagaacatcgtcgagtttctgaaccggtggatcaccttctgccagtccatcatctccacactgaccggcggcggaggaagcggtggcggcggtagcggaggtggtggttctggtggtggcggttctattacatgccctcctccaatgtccgtggaacacgccgacatctgggtcaagtcctacagcctgtactccagagagcggtacatctgcaactccggcttcaagagaaaggccggcacctctagcctgaccgagtgcgtgctgaacaaggccaccaatgtggcccactggacaacccctagcctgaagtgtattagaggtggcggaggatctggcggaggcggatctggatccgccgagtctaagtacggccctccttgtcctccatgtcctgctccagaagctgccggagggcccagtgtgtttctgttccctccaaagcctaaggaccagctgatgatctctcggacccctgaagtgacctgcgtggtggtggatgtgtcccaagaggaccctgaggtgcagttcaattggtacgtggacggcgtggaagtgcacaacgccaagaccaagcctagagaggaacagttcaactccacctacagagtggtgtccgtgctgaccgtgctgcaccaggattggctgaacggcaaagagtacaagtgcaaggtgtccaacaagggcctgccttccagcatcgaaaagaccatctccaaggccaagggccagcctagggaaccccaggtttacaccctgcctccaagccaagaggaaatgaccaagaaccaggtgtccctgacctgcctggtcaagggcttctacccttccgatatcgccgtggaatgggagagcaatggccagcctgagaacaactacaagaccacacctcctgtgctggactccgacggctccttctttctgtactcccgcctgaccgtggacaagtccagatggcaagagggcaacgtgttctcctgctctgtgctgcacgaggccctgcacaatcactacacccagaagtccctgtctctgtcccttggc

SEQ ID NO: 165 - DNA, 1359 bp, synthetic construct
  source 1..1359: mol_type = other DNA
gctcctacctcctccagcaccaagaaaacccagctgcagttggagcatctgctgctggacctgcagatgatcctgaacggctccatgcacatcgacgctaccctgtacaccgagtccgacgtgcacccttcctgtaaagtgaccgccatgaagtgctttctgctcgagctgcaagtgatctccctggaatccaagaacttccacctgaggccaagagagttcatctccgacatcaacctgatcgtgctggaactgaagggctccaacggcaacgtgaccgagtctggctgtaaagagtgcgaggaactggaagagaagaacatcgtcgagtttctgaaccggtggatcaccttctgccagtccatcatctccacactgaccggcggcggaggaagcggtggcggcggtagcggaggtggtggttctggtggtggcggttctattacatgccctcctccaatgtccgtggaacacgccgacatctgggtcaagtcctacagcctgtactccagagagcggtacatctgcaactccggcttcaagagaaaggccggcacctctagcctgaccgagtgcgtgctgaacaaggccaccaatgtggcccactggacaacccctagcctgaagtgtattagaggtggcggaggatctggcggaggcggatctggatccgccgagtctaagtacggccctccttgtcctccatgtcctgctccagaagctgccggagggcccagtgtgtttctgttccctccaaagcctaaggaccagctgatgatctctcggacccctgaagtgacctgcgtggtggtggatgtgtcccaagaggaccctgaggtgcagttcaattggtacgtggacggcgtggaagtgcacaacgccaagaccaagcctagagaggaacagttcaactccacctacagagtggtgtccgtgctgaccgtgctgcaccaggattggctgaacggcaaagagtacaagtgcaaggtgtccaacaagggcctgccttccagcatcgaaaagaccatctccaaggccaagggccagcctagggaaccccaggtttacaccctgcctccaagccaagaggaaatgaccaagaaccaggtgtccctgacctgcctggtcaagggcttctacccttccgatatcgccgtggaatgggagagcaatggccagcctgagaacaactacaagaccacacctcctgtgctggactccgacggctccttctttctgtactcccgcctgaccgtggacaagtccagatggcaagagggcaacgtgttctcctgctctgtgctgcacgaggccctgcacaatcactacacccagaagtccctgtctctgtcccttggc

SEQ ID NO: 166 - DNA, 1359 bp, synthetic construct
  source 1..1359: mol_type = other DNA
gctcctacctcctccagcaccaagaaaacccagctgcagttggagcatctgctgctggacctgcagatgatcctgaacggctccatgcacatcgacgctaccctgtacaccgagtccgacgtgcacccttcctgtaaagtgaccgccatgaagtgctttctgctcgagctgcaagtgatctccctggaatccaagaacttccacctgaggccaagagagttcatcgacaacatcaacctgatcgtcctggaactgaagggctccaacggcaacgtgaccgagtctggctgtaaagagtgcgaggaactggaagagaagaacatcgtcgagtttctgaaccggtggatcaccttctgccagtccatcatctccacactgaccggcggcggaggaagcggtggcggcggtagcggaggtggtggttctggtggtggcggttctattacatgccctcctccaatgtccgtggaacacgccgacatctgggtcaagtcctacagcctgtactccagagagcggtacatctgcaactccggcttcaagagaaaggccggcacctctagcctgaccgagtgcgtgctgaacaaggccaccaatgtggcccactggacaacccctagcctgaagtgtattagaggtggcggaggatctggcggaggcggatctggatccgccgagtctaagtacggccctccttgtcctccatgtcctgctccagaagctgccggagggcccagtgtgtttctgttccctccaaagcctaaggaccagctgatgatctctcggacccctgaagtgacctgcgtggtggtggatgtgtcccaagaggaccctgaggtgcagttcaattggtacgtggacggcgtggaagtgcacaacgccaagaccaagcctagagaggaacagttcaactccacctacagagtggtgtccgtgctgaccgtgctgcaccaggattggctgaacggcaaagagtacaagtgcaaggtgtccaacaagggcctgccttccagcatcgaaaagaccatctccaaggccaagggccagcctagggaaccccaggtttacaccctgcctccaagccaagaggaaatgaccaagaaccaggtgtccctgacctgcctggtcaagggcttctacccttccgatatcgccgtggaatgggagagcaatggccagcctgagaacaactacaagaccacacctcctgtgctggactccgacggctccttctttctgtactcccgcctgaccgtggacaagtccagatggcaagagggcaacgtgttctcctgctctgtgctgcacgaggccctgcacaatcactacacccagaagtccctgtctctgtcccttggc

SEQ ID NO: 167 - DNA, 1359 bp, synthetic construct
  source 1..1359: mol_type = other DNA
gctcctacctcctccagcaccaagaaaacccagctgcagttggagcatctgctgctggacctgcagatgatcctgaacggctccatgcacatcgacgctaccctgtacaccgagtccgacgtgcacccttcctgtaaagtgaccgccatgaagtgctttctgctcgagctgcaagtgatctccctggaatccaagaacttccacctgaggccaagagagttcatcgacgacatcaacgtgatcgtgctggaactgaagggctccaacggcaacgtgaccgagtctggctgtaaagagtgcgaggaactggaagagaagaacatcgtcgagtttctgaaccggtggatcaccttctgccagtccatcatctccacactgaccggcggcggaggaagcggtggcggcggtagcggaggtggtggttctggtggtggcggttctattacatgccctcctccaatgtccgtggaacacgccgacatctgggtcaagtcctacagcctgtactccagagagcggtacatctgcaactccggcttcaagagaaaggccggcacctctagcctgaccgagtgcgtgctgaacaaggccaccaatgtggcccactggacaacccctagcctgaagtgtattagaggtggcggaggatctggcggaggcggatctggatccgccgagtctaagtacggccctccttgtcctccatgtcctgctccagaagctgccggagggcccagtgtgtttctgttccctccaaagcctaaggaccagctgatgatctctcggacccctgaagtgacctgcgtggtggtggatgtgtcccaagaggaccctgaggtgcagttcaattggtacgtggacggcgtggaagtgcacaacgccaagaccaagcctagagaggaacagttcaactccacctacagagtggtgtccgtgctgaccgtgctgcaccaggattggctgaacggcaaagagtacaagtgcaaggtgtccaacaagggcctgccttccagcatcgaaaagaccatctccaaggccaagggccagcctagggaaccccaggtttacaccctgcctccaagccaagaggaaatgaccaagaaccaggtgtccctgacctgcctggtcaagggcttctacccttccgatatcgccgtggaatgggagagcaatggccagcctgagaacaactacaagaccacacctcctgtgctggactccgacggctccttctttctgtactcccgcctgaccgtggacaagtccagatggcaagagggcaacgtgttctcctgctctgtgctgcacgaggccctgcacaatcactacacccagaagtccctgtctctgtcccttggc

SEQ ID NO: 168 - DNA, 1359 bp, synthetic construct
  source 1..1359: mol_type = other DNA
gctcctacctcctccagcaccaagaaaacccagctgcagttggagcatctgctgctggacctgcagatgatcctgaacggctccatgcacatcgacgctaccctgtacaccgagtccgacgtgcacccttcctgtaaagtgaccgccatgaagtgctttctgctcgagctgcaagtgatctccctggaatccaagaacttccacctgaggccaagagagttcatcgacgacatcaacctgatcgtgctggaactgaagggctccaacggcaacgtgaccgagtctggctgtaaagagtgcgaggaactggaagagaagaacatcgtcgagtttctgaaccggtggatcaccttctgccagtccatcatctccacactgaccggcggcggaggaagcggtggcggcggtagcggaggtggtggttctggtggtggcggttctattacatgccctcctccaatgtccgtggaacacgccgacatctgggtcaagtcctacagcctgtactccagagagcggtacatctgcaactccggcttcaagagaaaggccggcacctctagcctgaccgagtgcgtgctgaacaaggccaccaatgtggcccactggacaacccctagcctgaagtgtattagaggtggcggaggatctggcggaggcggatctggatccgccgagtctaagtacggccctccttgtcctccatgtcctgctccagaagctgccggagggcccagtgtgtttctgttccctccaaagcctaaggaccagctgatgatctctcggacccctgaagtgacctgcgtggtggtggatgtgtcccaagaggaccctgaggtgcagttcaattggtacgtggacggcgtggaagtgcacaacgccaagaccaagcctagagaggaacagttcaactccacctacagagtggtgtccgtgctgaccgtgctgcaccaggattggctgaacggcaaagagtacaagtgcaaggtgtccaacaagggcctgccttccagcatcgaaaagaccatctccaaggccaagggccagcctagggaaccccaggtttacaccctgcctccaagccaagaggaaatgaccaagaaccaggtgtccctgacctgcctggtcaagggcttctacccttccgatatcgccgtggaatgggagagcaatggccagcctgagaacaactacaagaccacacctcctgtgctggactccgacggctccttctttctgtactcccgcctgaccgtggacaagtccagatggcaagagggcaacgtgttctcctgctctgtgctgcacgaggccctgcacaatcactacacccagaagtccctgtctctgtcccttggc

SEQ ID NO: 169 - DNA, 1359 bp, synthetic construct
  source 1..1359: mol_type = other DNA
gctcctacctcctccagcaccaagaaaacccagctgcagttggagcatctgctgctggacctgcagatgatcctgaacggctccatgcacatcgacgctaccctgtacaccgagtccgacgtgcacccttcctgtaaagtgaccgccatgaagtgctttctgttggagctgcaagtgatctccctggaatccaagaacttccacctgaggcctcgggacctgatcgaaaacatcaacgtgatcgtgctggaactgaagggctccaacggcaacgtgaccgagtctggctgtaaagagtgcgaggaactggaagagaagaacatcgtcgagtttctgaaccggtggatcaccttctgccagtccatcatctccacactgaccggcggcggaggaagcggtggcggcggtagcggaggtggtggttctggtggtggcggttctattacatgccctcctccaatgtccgtggaacacgccgacatctgggtcaagtcctacagcctgtactccagagagcggtacatctgcaactccggcttcaagagaaaggccggcacctctagcctgaccgagtgcgtgctgaacaaggccaccaatgtggcccactggacaacccctagcctgaagtgtattagaggtggcggaggatctggcggaggcggatctggatccgccgagtctaagtacggccctccttgtcctccatgtcctgctccagaagctgccggagggcccagtgtgtttctgttccctccaaagcctaaggaccagctgatgatctctcggacccctgaagtgacctgcgtggtggtggatgtgtcccaagaggaccctgaggtgcagttcaattggtacgtggacggcgtggaagtgcacaacgccaagaccaagcctagagaggaacagttcaactccacctacagagtggtgtccgtgctgaccgtgctgcaccaggattggctgaacggcaaagagtacaagtgcaaggtgtccaacaagggcctgccttccagcatcgaaaagaccatctccaaggccaagggccagcctagggaaccccaggtttacaccctgcctccaagccaagaggaaatgaccaagaaccaggtgtccctgacctgcctggtcaagggcttctacccttccgatatcgccgtggaatgggagagcaatggccagcctgagaacaactacaagaccacacctcctgtgctggactccgacggctccttctttctgtactcccgcctgaccgtggacaagtccagatggcaagagggcaacgtgttctcctgctctgtgctgcacgaggccctgcacaatcactacacccagaagtccctgtctctgtcccttggc

SEQ ID NO: 170 - DNA, 1359 bp, synthetic construct
  source 1..1359: mol_type = other DNA
gctcctacctcctccagcaccaagaaaacccagctgcagttggagcatctgctgctggacctgcagatgatcctgaacggctccatgcacatcgacgctaccctgtacaccgagtccgacgtgcacccttcctgtaaagtgaccgccatgaagtgctttctgttggagctgcaagtgatctccctggaatccaagaacttccacctgaggcctcgggacctgatcaacaacatcaacgtgatcgtgctggaactgaagggctccaacggcaacgtgaccgagtctggctgtaaagagtgcgaggaactggaagagaagaacatcgtcgagtttctgaaccggtggatcaccttctgccagtccatcatctccacactgaccggcggcggaggaagcggtggcggcggtagcggaggtggtggttctggtggtggcggttctattacatgccctcctccaatgtccgtggaacacgccgacatctgggtcaagtcctacagcctgtactccagagagcggtacatctgcaactccggcttcaagagaaaggccggcacctctagcctgaccgagtgcgtgctgaacaaggccaccaatgtggcccactggacaacccctagcctgaagtgtattagaggtggcggaggatctggcggaggcggatctggatccgccgagtctaagtacggccctccttgtcctccatgtcctgctccagaagctgccggagggcccagtgtgtttctgttccctccaaagcctaaggaccagctgatgatctctcggacccctgaagtgacctgcgtggtggtggatgtgtcccaagaggaccctgaggtgcagttcaattggtacgtggacggcgtggaagtgcacaacgccaagaccaagcctagagaggaacagttcaactccacctacagagtggtgtccgtgctgaccgtgctgcaccaggattggctgaacggcaaagagtacaagtgcaaggtgtccaacaagggcctgccttccagcatcgaaaagaccatctccaaggccaagggccagcctagggaaccccaggtttacaccctgcctccaagccaagaggaaatgaccaagaaccaggtgtccctgacctgcctggtcaagggcttctacccttccgatatcgccgtggaatgggagagcaatggccagcctgagaacaactacaagaccacacctcctgtgctggactccgacggctccttctttctgtactcccgcctgaccgtggacaagtccagatggcaagagggcaacgtgttctcctgctctgtgctgcacgaggccctgcacaatcactacacccagaagtccctgtctctgtcccttggc

SEQ ID NO: 171 - DNA, 1359 bp, synthetic construct
  source 1..1359: mol_type = other DNA
gctcctacctcctccagcaccaagaaaacccagctgcagttggagcatctgctgctggacctgcagatgatcctgaacggctccatgcacatcgacgctaccctgtacaccgagtccgacgtgcacccttcctgtaaagtgaccgccatgaagtgctttctgttggagctgcaagtgatctccctggaatccaagaacttccacctgaggcctcgggacctgatcaagaacatcaacgtgatcgtgctggaactgaagggctccaacggcaacgtgaccgagtctggctgtaaagagtgcgaggaactggaagagaagaacatcgtcgagtttctgaaccggtggatcaccttctgccagtccatcatctccacactgaccggcggcggaggaagcggtggcggcggtagcggaggtggtggttctggtggtggcggttctattacatgccctcctccaatgtccgtggaacacgccgacatctgggtcaagtcctacagcctgtactccagagagcggtacatctgcaactccggcttcaagagaaaggccggcacctctagcctgaccgagtgcgtgctgaacaaggccaccaatgtggcccactggacaacccctagcctgaagtgtattagaggtggcggaggatctggcggaggcggatctggatccgccgagtctaagtacggccctccttgtcctccatgtcctgctccagaagctgccggagggcccagtgtgtttctgttccctccaaagcctaaggaccagctgatgatctctcggacccctgaagtgacctgcgtggtggtggatgtgtcccaagaggaccctgaggtgcagttcaattggtacgtggacggcgtggaagtgcacaacgccaagaccaagcctagagaggaacagttcaactccacctacagagtggtgtccgtgctgaccgtgctgcaccaggattggctgaacggcaaagagtacaagtgcaaggtgtccaacaagggcctgccttccagcatcgaaaagaccatctccaaggccaagggccagcctagggaaccccaggtttacaccctgcctccaagccaagaggaaatgaccaagaaccaggtgtccctgacctgcctggtcaagggcttctacccttccgatatcgccgtggaatgggagagcaatggccagcctgagaacaactacaagaccacacctcctgtgctggactccgacggctccttctttctgtactcccgcctgaccgtggacaagtccagatggcaagagggcaacgtgttctcctgctctgtgctgcacgaggccctgcacaatcactacacccagaagtccctgtctctgtcccttggc

SEQ ID NO: 172 - DNA, 1359 bp, synthetic construct
  source 1..1359: mol_type = other DNA
gctcctacctcctccagcaccaagaaaacccagctgcagttggagcatctgctgctggacctgcagatgatcctgaacggctccatgcacatcgacgctaccctgtacaccgagtccgacgtgcacccttcctgtaaagtgaccgccatgaagtgctttctgttggagctgcaagtgatctccctggaatccaagaacttccacctgaggcctcgggacctgatcctcaacatcaacgtgatcgtgctggaactgaagggctccaacggcaacgtgaccgagtctggctgtaaagagtgcgaggaactggaagagaagaacatcgtcgagtttctgaaccggtggatcaccttctgccagtccatcatctccacactgaccggcggcggaggaagcggtggcggcggtagcggaggtggtggttctggtggtggcggttctattacatgccctcctccaatgtccgtggaacacgccgacatctgggtcaagtcctacagcctgtactccagagagcggtacatctgcaactccggcttcaagagaaaggccggcacctctagcctgaccgagtgcgtgctgaacaaggccaccaatgtggcccactggacaacccctagcctgaagtgtattagaggtggcggaggatctggcggaggcggatctggatccgccgagtctaagtacggccctccttgtcctccatgtcctgctccagaagctgccggagggcccagtgtgtttctgttccctccaaagcctaaggaccagctgatgatctctcggacccctgaagtgacctgcgtggtggtggatgtgtcccaagaggaccctgaggtgcagttcaattggtacgtggacggcgtggaagtgcacaacgccaagaccaagcctagagaggaacagttcaactccacctacagagtggtgtccgtgctgaccgtgctgcaccaggattggctgaacggcaaagagtacaagtgcaaggtgtccaacaagggcctgccttccagcatcgaaaagaccatctccaaggccaagggccagcctagggaaccccaggtttacaccctgcctccaagccaagaggaaatgaccaagaaccaggtgtccctgacctgcctggtcaagggcttctacccttccgatatcgccgtggaatgggagagcaatggccagcctgagaacaactacaagaccacacctcctgtgctggactccgacggctccttctttctgtactcccgcctgaccgtggacaagtccagatggcaagagggcaacgtgttctcctgctctgtgctgcacgaggccctgcacaatcactacacccagaagtccctgtctctgtcccttggc

SEQ ID NO: 173 - DNA, 1359 bp, synthetic construct
  source 1..1359: mol_type = other DNA
gctcctacctcctccagcaccaagaaaacccagctgcagttggagcatctgctgctggacctgcagatgatcctgaacggctccatgcacatcgacgctaccctgtacaccgagtccgacgtgcacccttcctgtaaagtgaccgccatgaagtgctttctgctcgagctgcaagtgatctccctggaatccaagaacttccacctgaggcctcgggacttcatcgacaacatcaacgtgatcgtgctggaactgaagggctccaacggcaacgtgaccgagtctggctgtaaagagtgcgaggaactggaagagaagaacatcgtcgagtttctgaaccggtggatcaccttctgccagtccatcatctccacactgaccggcggcggaggaagcggtggcggcggtagcggaggtggtggttctggtggtggcggttctattacatgccctcctccaatgtccgtggaacacgccgacatctgggtcaagtcctacagcctgtactccagagagcggtacatctgcaactccggcttcaagagaaaggccggcacctctagcctgaccgagtgcgtgctgaacaaggccaccaatgtggcccactggacaacccctagcctgaagtgtattagaggtggcggaggatctggcggaggcggatctggatccgccgagtctaagtacggccctccttgtcctccatgtcctgctccagaagctgccggagggcccagtgtgtttctgttccctccaaagcctaaggaccagctgatgatctctcggacccctgaagtgacctgcgtggtggtggatgtgtcccaagaggaccctgaggtgcagttcaattggtacgtggacggcgtggaagtgcacaacgccaagaccaagcctagagaggaacagttcaactccacctacagagtggtgtccgtgctgaccgtgctgcaccaggattggctgaacggcaaagagtacaagtgcaaggtgtccaacaagggcctgccttccagcatcgaaaagaccatctccaaggccaagggccagcctagggaaccccaggtttacaccctgcctccaagccaagaggaaatgaccaagaaccaggtgtccctgacctgcctggtcaagggcttctacccttccgatatcgccgtggaatgggagagcaatggccagcctgagaacaactacaagaccacacctcctgtgctggactccgacggctccttctttctgtactcccgcctgaccgtggacaagtccagatggcaagagggcaacgtgttctcctgctctgtgctgcacgaggccctgcacaatcactacacccagaagtccctgtctctgtcccttggc

SEQ ID NO: 174 - DNA, 1359 bp, synthetic construct
  source 1..1359: mol_type = other DNA
gctcctacctcctccagcaccaagaaaacccagctgcagttggagcatctgctgctggacctgcagatgatcctgaacggctccatgcacatcgacgctaccctgtacaccgagtccgacgtgcacccttcctgtaaagtgaccgccatgaagtgctttctgctcgagctgcaagtgatctccctggaatccaagaacttccacctgaggcctcgggacctgatcgacgacatcaacgtgatcgtgctggaactgaagggctccaacggcaacgtgaccgagtctggctgtaaagagtgcgaggaactggaagagaagaacatcgtcgagtttctgaaccggtggatcaccttctgccagtccatcatctccacactgaccggcggcggaggaagcggtggcggcggtagcggaggtggtggttctggtggtggcggttctattacatgccctcctccaatgtccgtggaacacgccgacatctgggtcaagtcctacagcctgtactccagagagcggtacatctgcaactccggcttcaagagaaaggccggcacctctagcctgaccgagtgcgtgctgaacaaggccaccaatgtggcccactggacaacccctagcctgaagtgtattagaggtggcggaggatctggcggaggcggatctggatccgccgagtctaagtacggccctccttgtcctccatgtcctgctccagaagctgccggagggcccagtgtgtttctgttccctccaaagcctaaggaccagctgatgatctctcggacccctgaagtgacctgcgtggtggtggatgtgtcccaagaggaccctgaggtgcagttcaattggtacgtggacggcgtggaagtgcacaacgccaagaccaagcctagagaggaacagttcaactccacctacagagtggtgtccgtgctgaccgtgctgcaccaggattggctgaacggcaaagagtacaagtgcaaggtgtccaacaagggcctgccttccagcatcgaaaagaccatctccaaggccaagggccagcctagggaaccccaggtttacaccctgcctccaagccaagaggaaatgaccaagaaccaggtgtccctgacctgcctggtcaagggcttctacccttccgatatcgccgtggaatgggagagcaatggccagcctgagaacaactacaagaccacacctcctgtgctggactccgacggctccttctttctgtactcccgcctgaccgtggacaagtccagatggcaagagggcaacgtgttctcctgctctgtgctgcacgaggccctgcacaatcactacacccagaagtccctgtctctgtcccttggc

SEQ ID NO: 175 - DNA, 1359 bp, synthetic construct
  source 1..1359: mol_type = other DNA
gctcctacctcctccagcaccaagaaaacccagctgcagttggagcatctgctgctggacctgcagatgatcctgaacggctccatgcacatcgacgctaccctgtacaccgagtccgacgtgcacccttcctgtaaagtgaccgccatgaagtgctttctgctcgagctgcaagtgatctccctggaatccaagaacttccacctgaggcctcgggacctgatcgacaacatcaacctgatcgtgctggaactgaagggctccaacggcaacgtgaccgagtctggctgtaaagagtgcgaggaactggaagagaagaacatcgtcgagtttctgaaccggtggatcaccttctgccagtccatcatctccacactgaccggcggcggaggaagcggtggcggcggtagcggaggtggtggttctggtggtggcggttctattacatgccctcctccaatgtccgtggaacacgccgacatctgggtcaagtcctacagcctgtactccagagagcggtacatctgcaactccggcttcaagagaaaggccggcacctctagcctgaccgagtgcgtgctgaacaaggccaccaatgtggcccactggacaacccctagcctgaagtgtattagaggtggcggaggatctggcggaggcggatctggatccgccgagtctaagtacggccctccttgtcctccatgtcctgctccagaagctgccggagggcccagtgtgtttctgttccctccaaagcctaaggaccagctgatgatctctcggacccctgaagtgacctgcgtggtggtggatgtgtcccaagaggaccctgaggtgcagttcaattggtacgtggacggcgtggaagtgcacaacgccaagaccaagcctagagaggaacagttcaactccacctacagagtggtgtccgtgctgaccgtgctgcaccaggattggctgaacggcaaagagtacaagtgcaaggtgtccaacaagggcctgccttccagcatcgaaaagaccatctccaaggccaagggccagcctagggaaccccaggtttacaccctgcctccaagccaagaggaaatgaccaagaaccaggtgtccctgacctgcctggtcaagggcttctacccttccgatatcgccgtggaatgggagagcaatggccagcctgagaacaactacaagaccacacctcctgtgctggactccgacggctccttctttctgtactcccgcctgaccgtggacaagtccagatggcaagagggcaacgtgttctcctgctctgtgctgcacgaggccctgcacaatcactacacccagaagtccctgtctctgtcccttggc

SEQ ID NO: 176 - DNA, 1359 bp, synthetic construct
  source 1..1359: mol_type = other DNA
gctcctacctcctccagcaccaagaaaacccagctgcagttggagcatctgctgctggacctgcagatgatcctgaacggctccatgcacatcgacgctaccctgtacaccgagtccgacgtgcacccttcctgtaaagtgaccgccatgaagtgctttctgctcgagctgcaagtgatctccctggaatccaagaacttccacctgaggcctcgggacttcatcgacgacatcaacgtgatcgtgctggaactgaagggctccaacggcaacgtgaccgagtctggctgtaaagagtgcgaggaactggaagagaagaacatcgtcgagtttctgaaccggtggatcaccttctgccagtccatcatctccacactgaccggcggcggaggaagcggtggcggcggtagcggaggtggtggttctggtggtggcggttctattacatgccctcctccaatgtccgtggaacacgccgacatctgggtcaagtcctacagcctgtactccagagagcggtacatctgcaactccggcttcaagagaaaggccggcacctctagcctgaccgagtgcgtgctgaacaaggccaccaatgtggcccactggacaacccctagcctgaagtgtattagaggtggcggaggatctggcggaggcggatctggatccgccgagtctaagtacggccctccttgtcctccatgtcctgctccagaagctgccggagggcccagtgtgtttctgttccctccaaagcctaaggaccagctgatgatctctcggacccctgaagtgacctgcgtggtggtggatgtgtcccaagaggaccctgaggtgcagttcaattggtacgtggacggcgtggaagtgcacaacgccaagaccaagcctagagaggaacagttcaactccacctacagagtggtgtccgtgctgaccgtgctgcaccaggattggctgaacggcaaagagtacaagtgcaaggtgtccaacaagggcctgccttccagcatcgaaaagaccatctccaaggccaagggccagcctagggaaccccaggtttacaccctgcctccaagccaagaggaaatgaccaagaaccaggtgtccctgacctgcctggtcaagggcttctacccttccgatatcgccgtggaatgggagagcaatggccagcctgagaacaactacaagaccacacctcctgtgctggactccgacggctccttctttctgtactcccgcctgaccgtggacaagtccagatggcaagagggcaacgtgttctcctgctctgtgctgcacgaggccctgcacaatcactacacccagaagtccctgtctctgtcccttggc

SEQ ID NO: 177 - DNA, 1359 bp, synthetic construct
  source 1..1359: mol_type = other DNA
gctcctacctcctccagcaccaagaaaacccagctgcagttggagcatctgctgctggacctgcagatgatcctgaacggctccatgcacatcgacgctaccctgtacaccgagtccgacgtgcacccttcctgtaaagtgaccgccatgaagtgctttctgctcgagctgcaagtgatctccctggaatccaagaacttccacctgaggcctcgggacctgatcgacgacatcaacctgatcgtgctggaactgaagggctccaacggcaacgtgaccgagtctggctgtaaagagtgcgaggaactggaagagaagaacatcgtcgagtttctgaaccggtggatcaccttctgccagtccatcatctccacactgaccggcggcggaggaagcggtggcggcggtagcggaggtggtggttctggtggtggcggttctattacatgccctcctccaatgtccgtggaacacgccgacatctgggtcaagtcctacagcctgtactccagagagcggtacatctgcaactccggcttcaagagaaaggccggcacctctagcctgaccgagtgcgtgctgaacaaggccaccaatgtggcccactggacaacccctagcctgaagtgtattagaggtggcggaggatctggcggaggcggatctggatccgccgagtctaagtacggccctccttgtcctccatgtcctgctccagaagctgccggagggcccagtgtgtttctgttccctccaaagcctaaggaccagctgatgatctctcggacccctgaagtgacctgcgtggtggtggatgtgtcccaagaggaccctgaggtgcagttcaattggtacgtggacggcgtggaagtgcacaacgccaagaccaagcctagagaggaacagttcaactccacctacagagtggtgtccgtgctgaccgtgctgcaccaggattggctgaacggcaaagagtacaagtgcaaggtgtccaacaagggcctgccttccagcatcgaaaagaccatctccaaggccaagggccagcctagggaaccccaggtttacaccctgcctccaagccaagaggaaatgaccaagaaccaggtgtccctgacctgcctggtcaagggcttctacccttccgatatcgccgtggaatgggagagcaatggccagcctgagaacaactacaagaccacacctcctgtgctggactccgacggctccttctttctgtactcccgcctgaccgtggacaagtccagatggcaagagggcaacgtgttctcctgctctgtgctgcacgaggccctgcacaatcactacacccagaagtccctgtctctgtcccttggc

SEQ ID NO: 178 - DNA, 1359 bp, synthetic construct
  source 1..1359: mol_type = other DNA
gctcctacctcctccagcaccaagaaaacccagctgcagttggagcatctgctgctggacctgcagatgatcctgaacggctccatgcacatcgacgctaccctgtacaccgagtccgacgtgcacccttcctgtaaagtgaccgccatgaagtgctttctgctcgagctgcaagtgatctccctggaatccaagaacttccacctgaggcctcgggacttcatcgacaacatcaacctgatcgtgctggaactgaagggctccaacggcaacgtgaccgagtctggctgtaaagagtgcgaggaactggaagagaagaacatcgtcgagtttctgaaccggtggatcaccttctgccagtccatcatctccacactgaccggcggcggaggaagcggtggcggcggtagcggaggtggtggttctggtggtggcggttctattacatgccctcctccaatgtccgtggaacacgccgacatctgggtcaagtcctacagcctgtactccagagagcggtacatctgcaactccggcttcaagagaaaggccggcacctctagcctgaccgagtgcgtgctgaacaaggccaccaatgtggcccactggacaacccctagcctgaagtgtattagaggtggcggaggatctggcggaggcggatctggatccgccgagtctaagtacggccctccttgtcctccatgtcctgctccagaagctgccggagggcccagtgtgtttctgttccctccaaagcctaaggaccagctgatgatctctcggacccctgaagtgacctgcgtggtggtggatgtgtcccaagaggaccctgaggtgcagttcaattggtacgtggacggcgtggaagtgcacaacgccaagaccaagcctagagaggaacagttcaactccacctacagagtggtgtccgtgctgaccgtgctgcaccaggattggctgaacggcaaagagtacaagtgcaaggtgtccaacaagggcctgccttccagcatcgaaaagaccatctccaaggccaagggccagcctagggaaccccaggtttacaccctgcctccaagccaagaggaaatgaccaagaaccaggtgtccctgacctgcctggtcaagggcttctacccttccgatatcgccgtggaatgggagagcaatggccagcctgagaacaactacaagaccacacctcctgtgctggactccgacggctccttctttctgtactcccgcctgaccgtggacaagtccagatggcaagagggcaacgtgttctcctgctctgtgctgcacgaggccctgcacaatcactacacccagaagtccctgtctctgtcccttggc

SEQ ID NO: 179 - DNA, 1101 bp, synthetic construct
  source 1..1101: mol_type = other DNA
gccgagtctaagtacggacctccttgtcctccatgtcctgctccagaagctgctggcggcccttccgtgtttctgttccctccaaagcctaaggacaccctgatgatctctcggacccctgaagtgacctgcgtggtggtggatgtgtcccaagaggatcccgaggtgcagttcaattggtacgtggacggcgtggaagtgcacaacgccaagaccaagcctagagaggaacagttcaactccacctacagagtggtgtccgtgctgaccgtgctgcaccaggattggctgaacggcaaagagtacaagtgcaaggtgtccaacaagggcctgccttccagcatcgaaaagaccatctccaaggccaagggccagcctagggaaccccaggtttacaccctgcctccaagccaagaggaaatgaccaagaaccaggtgtccctgacctgcctggtcaagggcttctacccttccgatatcgccgtggaatgggagagcaatggccagcctgagaacaactacaagaccacacctcctgtgctggactccgacggctccttctttctgtactcccgcctgaccgtggacaagtccagatggcaagagggcaacgtgttctcctgctccgtgatgcacgaggccctgcacaatcactacacccagaagtccctgtctctgtcccttggaggtggcggaggatctgctcctacctcctccagcaccaagaaaacccagctgcagttggagcatctgctgctggacctgcagatgatcctgaatggcatcaacaattacaagaaccccaagctgacccggatgctgaccttcaagttctacatgcccaagaaggccaccgagctgaaacatctgcagtgcctggaagaggaactgaagcccctggaagaagtgctgaatctggcccagtccaagaacttccacctgaggcctcgggacctgatctccaacatcaacgtgatcgtgctcgagctgaagggctccgagacaaccttcatgtgcgagtacgccgacgagacagctaccatcgtggaatttctgaaccggtggatcaccttctgccagtccatcatcagcaccctgacc

SEQ ID NO: 180 - protein, 18 aa, synthetic construct
MDWTWILFLVAAATRVHS

SEQ ID NO: 181 - DNA, 54 bp, synthetic construct
  source 1..54: mol_type = other DNA
atggattggacatggatactctttcttgttgccgcagccacgcgagtccattcc

SEQ ID NO: 182 - DNA, 48 bp, synthetic construct
  source 1..48: mol_type = other DNA
gagttacctacccagggaacattttcaaatgtttctacaaatgtatcc

SEQ ID NO: 183 - protein, 386 aa, synthetic construct
GIHVFILGCFSAGLPKTEANWVNVISDLKKIEDLIQSMHIDATLYTESDVHPSCKVTAMKCFLLELQVISLESGDASIHDTVENLIILANNSLSSNGNVTESGCKECEELEEKNIKEFLQSFVHIVQMFINTSELPTQGTFSNVSTNVSITCPPPMSVEHADIWVKSYSLYSRERYICNSGFKRKAGTSSLTECVLNKATNVAHWTTPSLKCIRDPALVHQRPAPPSTVTTAGVTPQPESLSPSGKEPAASSPSSNNTAATTAAIVPGSQLMPSKSPSTGTTEISSHESSHGTPSQTTAKNWELTASASHQPPGVYPQGHSDTTVAISTSTVLLCGLSAVSLLACYLKSRQTPPLASVEMEAMEALPVTWGTSSRDEDLENCSHHL

SEQ ID NO: 184 - DNA, 1161 bp, synthetic construct
  source 1..1161: mol_type = other DNA
ggcatccacgtgttcattctgggatgcttcagcgcaggcctgcctaaaaccgaggcgaactgggttaacgtgatcagcgatttgaaaaagattgaggatctgatccagtccatgcatattgacgcaaccttgtacacagagtcagatgtgcacccttcctgcaaagttacggctatgaagtgttttttgcttgaattgcaagtaataagtttggagtctggcgatgcatctatacatgataccgtagaaaatttgatcatcctggctaataatagtttgtccagtaatggtaacgtaacagagagcggttgtaaagagtgtgaagagctcgaggaaaagaatataaaagaattcttgcaatcctttgtacatatcgtgcaaatgttcattaatacaagcgagttacctacccagggaacattttcaaatgtttctacaaatgtatccattacttgtccaccaccaatgtctgttgagcatgctgatatttgggtgaaatcttattctctctatagccgggaacgctatatctgcaattcaggatttaaaagaaaggctggtacctcttccttgaccgaatgtgtactgaataaagctacaaacgtggcacattggaccacgcctagccttaagtgtataagggaccccgcattagtgcatcagagacctgcacccccgagcaccgtgacaactgccggtgtcactcctcaacctgaatctctttctcccagcggtaaggaaccagctgccagtagtccgtcaagtaataataccgcagctactactgccgccatcgttcccgggtctcaactcatgccaagcaagagcccctcaaccgggacaaccgaaatttcctctcacgaaagttctcatgggactccaagccaaaccaccgctaagaattgggagttgaccgcctcagcaagtcatcaacccccaggggtatacccccaagggcattccgatactaccgttgcaattagcacttctacggtgttactttgcggattatctgcagtatccctgttggcctgttatcttaaaagccgtcagacaccgccactcgcttccgtcgagatggaagctatggaagcccttcccgtaacctggggcactagttcccgcgacgaggatctggagaattgtagtcatcatttgtaa

SEQ ID NO: 185 - protein, 380 aa, synthetic construct
APTSSSTKKTQLQLEHLLLDLQMILNGSMHIDATLYTESDVHPSCKVTAMKCFLLELQVISLESKNFHLRPRDLIDNINVIVLELKGSNGNVTESGCKECEELEEKNIVEFLNRWITFCQSIISTLTELPTQGTFSNVSTNVSITCPPPMSVEHADIWVKSYSLYSRERYICNSGFKRKAGTSSLTECVLNKATNVAHWTTPSLKCIRDPALVHQRPAPPSTVTTAGVTPQPESLSPSGKEPAASSPSSNNTAATTAAIVPGSQLMPSKSPSTGTTEISSHESSHGTPSQTTAKNWELTASASHQPPGVYPQGHSDTTVAISTSTVLLCGLSAVSLLACYLKSRQTPPLASVEMEAMEALPVTWGTSSRDEDLENCSHHL

SEQ ID NO: 186 - DNA, 1197 bp, synthetic construct
  source 1..1197: mol_type = other DNA
atggattggacatggatactctttcttgttgccgcagccacgcgagtccattccgctcccacaagttcaagtactaaaaaaacccaactgcaactggagcatttgcttttggatctccaaatgattctgaatggctcaatgcacattgacgctactctttacacagagagtgatgtacacccttcttgcaaggttaccgctatgaaatgctttctcttggaactccaagtaatcagtcttgaatctaaaaattttcatttgcgcccacgcgatctgatagacaacatcaacgtgatagtactggaactcaagggaagcaatggaaacgtcacagaatcaggttgtaaagaatgtgaggaattggaagaaaagaatatagtcgagttcctcaatcgctggatcactttttgccaatccattatatccactctgacagagttacctacccagggaacattttcaaatgtttctacaaatgtatccattacttgtccaccaccaatgtctgttgagcatgctgatatttgggtgaaatcttattctctctatagccgggaacgctatatctgcaattcaggatttaaaagaaaggctggtacctcttccttgaccgaatgtgtactgaataaagctacaaacgtggcacattggaccacgcctagccttaagtgtataagggaccccgcattagtgcatcagagacctgcacccccgagcaccgtgacaactgccggtgtcactcctcaacctgaatctctttctcccagcggtaaggaaccagctgccagtagtccgtcaagtaataataccgcagctactactgccgccatcgttcccgggtctcaactcatgccaagcaagagcccctcaaccgggacaaccgaaatttcctctcacgaaagttctcatgggactccaagccaaaccaccgctaagaattgggagttgaccgcctcagcaagtcatcaacccccaggggtatacccccaagggcattccgatactaccgttgcaattagcacttctacggtgttactttgcggattatctgcagtatccctgttggcctgttatcttaaaagccgtcagacaccgccactcgcttccgtcgagatggaagctatggaagcccttcccgtaacctggggcactagttcccgcgacgaggatctggagaattgtagtcatcatttgtaa